European Patent Application EP 4 726 047 A1, published April 15, 2026. Title: Method for producing 4-(aminomethyl)cyclohexane-1-carboxylic acid. Applicant: キリンホールディングス株式会社. The sequence listing filed with the application follows.

SEQUENCE LISTING (210 sequences)

SEQ ID NO: 1 - protein, 453 aa, Pseudomonas putida KT2440
MSVNNPQTREWQTLSGEHHLAPFSDYKQLKEKGPRIITKAQGVHLWDSEGHKILDGMAGLWCVAVGYGREELVQAAEKQMRELPYYNLFFQTAHPPALELAKAITDVAPKGMTHVFFTGSGSEGNDTVLRMVRHYWALKGKPHKQTIIGRINGYHGSTFAGACLGGMSGMHEQGGLPIPGIVHIPQPYWFGEGGDMTPDEFGVWAAEQLEKKILEVGEDNVAAFIAEPIQGAGGVIIPPETYWPKVKEILARYDILFVADEVICGFGRTGEWFGSDYYDLKPDLMTIAKGLTSGYIPMGGVIVRDTVAKVISEGGDFNHGFTYSGHPVAAAVGLENLRILRDEKIVEKARTEAAPYLQKRLRELQDHPLVGEVRGLGMLGAIELVKDKATRSRYEGKGVGMICRTFCFENGLIMRAVGDTMIIAPPLVISHAEIDELVEKARKCLDLTLEAIQ

SEQ ID NO: 2 - protein, 460 aa, Pseudomonas putida KT2440
MNAPFAPQRQTRDYQAADAAHHIHAFLDQKALNAEGPRVIVGGERLHLWDSEGKRYLDGMSGLWCTQLGYGRRDLTAAAATQMDQLAYYNMFFHTTHPAVIELSELLFSLLPGHYSHAIYTNSGSEANEVLIRTVRRYWQVVGQPGKKIMIGRWNGYHGSTLAATALGGMKFMHDMGGLIPDVAHIDEPYWYAEGGELTPAEFGRRCALQLEEKILELGAENVAGFIAEPFQGAGGMIFPPESYWPEIQRICRQYDVLLCADEVIGGFGRTGEWFAHEYFGFEPDTLSIAKGLTSGYVPMGGLVLSKRIAEALVERGGVFAHGLTYSGHPVAAAVAIANLKALRDEGIVRQVKDDTGPYLQRILREVFADHPLIGQVQGAGLVAALQFAEHKPTRKRFANENDLAWQCRTFGFEEGVIIRSTLGRMIMAPALIANHSELDELVEKTRIAVDRTARLVGKL

SEQ ID NO: 3 - protein, 453 aa, Aeromonas salmonicida subsp. salmonicida
MQHTTREWQQLDASHHLHPFTDFQALNQKGSRIITRAEGIYLEDSDGRRILDGMAGLWCVNMGYGRQELVEAATKQMQQLPYYNLFFQTAHPPVIELATLLAEVTPSHLNHVFFTGSGSECNDTVLRMVRHYWASKGQPDKQVIISRHNAYHGSTVAGASLGGMKGMHAQGGLPIPGIVHIDQPYHFGEGQGMSAHEFGLERARQLEQKILELGVDKVAAFIGEPIQGAGGVIIPPDSYWPEIQRICDKYGILLIADEVICGFGRTGHWFASEGFGIKPDLMCLAKGITSGYLPMGAVMVGDRVARVLVEEGGEFNHGFTYSGHPVACAVAIANIKLMQSESIVKRIHDTIGPYLQRRWRELADHPLVGETRGKGLVAALEIVQDKQTNSRFPAGLQAGMTCREFCFNNGLVMRAVGDTMIISPPLVITEEQVDELVNLARLSLDLTAAKLKG

SEQ ID NO: 4 - protein, 459 aa, Escherichia coli K12 MG1655
MNRLPSSASALACSAHALNLIEKRTLDHEEMKALNREVIEYFKEHVNPGFLEYRKSVTAGGDYGAVEWQAGSLNTLVDTQGQEFIDCLGGFGIFNVGHRNPVVVSAVQNQLAKQPLHSQELLDPLRAMLAKTLAALTPGKLKYSFFCNSGTESVEAALKLAKAYQSPRGKFTFIATSGAFHGKSLGALSATAKSTFRKPFMPLLPGFRHVPFGNIEAMRTALNECKKTGDDVAAVILEPIQGEGGVILPPPGYLTAVRKLCDEFGALMILDEVQTGMGRTGKMFACEHENVQPDILCLAKALGGGVMPIGATIATEEVFSVLFDNPFLHTTTFGGNPLACAAALATINVLLEQNLPAQAEQKGDMLLDGFRQLAREYPDLVQEARGKGMLMAIEFVDNEIGYNFASEMFRQRVLVAGTLNNAKTIRIEPPLTLTIEQCELVIKAARKALAAMRVSVEEA

SEQ ID NO: 5 - DNA, 1362 bp, Pseudomonas putida KT2440
  source 1..1362: mol_type = genomic DNA
atgagcgtcaacaacccgcaaacccgtgaatggcaaaccctgagcggggagcatcacctcgcacctttcagtgactacaagcagctgaaggagaaggggccgcgcatcatcaccaaggcccagggtgtgcatttgtgggatagcgaggggcacaagatcctcgacggcatggccggtctatggtgcgtggcggtcggctacggacgtgaagagctggtgcaggcggcggaaaaacagatgcgcgagctgccgtactacaacctgttcttccagaccgctcacccgcctgcgctcgagctggccaaggcgatcaccgacgtggcgccgaaaggtatgacccatgtgttcttcaccggctccggctccgaaggcaacgacactgtgctgcgcatggtgcgtcactactgggcgctgaagggcaaaccgcacaagcagaccatcatcggccgcatcaacggttaccacggctccaccttcgccggtgcatgcctgggcggtatgagcggcatgcacgagcagggtggcctgccgatcccgggcatcgtgcacatccctcagccgtactggttcggcgagggaggcgacatgacccctgacgaattcggtgtctgggccgccgagcagttggagaagaagatcctcgaagtcggcgaagacaacgtcgcggccttcatcgccgagccgatccagggcgctggtggcgtgatcatcccgccggaaacctactggccgaaggtgaaggagatcctcgccaggtacgacatcctgttcgtcgccgacgaggtgatctgcggcttcggccgtaccggcgagtggttcggctcggactactacgacctcaagcccgacctgatgaccatcgcgaaaggcctgacctccggttacatccccatgggcggtgtgatcgtgcgtgacaccgtggccaaggtgatcagcgaaggcggcgacttcaaccacggtttcacctactccggccacccggtggcggccgcggtgggcctggaaaacctgcgcattctgcgtgacgagaaaattgtcgagaaggcgcgcacggaagcggcaccgtatttgcaaaagcgtttgcgcgagctgcaagaccatccactggtgggtgaagtgcgcggcctgggcatgctgggagcgatcgagctggtcaaggacaaggcaacccgcagccgttacgagggcaagggcgttggcatgatctgtcgcaccttctgcttcgagaacggcctgatcatgcgtgcggtgggtgacaccatgatcatcgcgccgccgctggtaatcagccatgcggagatcgacgaactggtggaaaaggcgcgcaagtgcctggacctgacccttgaggcgattcaataa

SEQ ID NO: 6 - DNA, 1383 bp, Pseudomonas putida KT2440
  source 1..1383: mol_type = genomic DNA
atgaacgcgcctttcgccccgcaacgccagacccgtgactaccaggcagccgatgccgcccaccacattcatgccttcctcgaccagaaggcgctgaacgccgaagggccgcgggtgatcgtcggtggcgaacgcctgcacctgtgggacagcgagggcaagcgttacctggatggcatgtccggcctgtggtgcacccagctcggttatggccgtcgtgacctgacggccgccgcggccacgcagatggatcagctggcctactacaacatgtttttccacaccacccacccggcggtgatcgaactgtccgagttgctgttcagcctgctgccggggcactacagccacgcgatctacaccaactccggctccgaggccaacgaggtactgatccgcaccgtgcgccgctactggcaggtggttggccagccaggcaagaaaatcatgatcggccgctggaacggctaccacggctcgaccctggcggccacggcgctgggtgggatgaagttcatgcacgacatgggcgggttgattccggatgtggcacacatcgacgaaccctactggtacgccgagggcggtgaactgactccggccgagttcggccgccgctgcgccctgcagctggaggaaaaaatcctcgaactgggtgccgagaacgttgccggcttcattgccgaacccttccagggggccggcggcatgatcttcccgccggaaagctactggccggaaatccagcgtatctgccgccagtacgacgtgctgctgtgcgccgatgaggtgatcggtggctttggccgcaccggcgaatggttcgcccatgaatacttcggcttcgagcccgacaccttgtcgattgccaagggcctgaccagcggctatgtgcccatgggcggcctggtgctgagcaagcgcattgccgaggcgttggtggagcgcggcggggtatttgcccacggcctgacctattccggccacccggtggcggcggcagtggccatcgccaacctgaaggcgctgcgtgacgaaggcatcgtgcgccaggtgaaggacgacacggggccgtacctgcagcgcatcctgcgggaagtgtttgccgaccacccattgatcggccaggtgcaaggggccgggctggtggcggcgctgcagttcgccgagcacaagccgacgcgcaagcgctttgccaacgagaacgacctggcctggcagtgccgcacctttggtttcgaggaaggggtgatcattcgctcgaccctgggccggatgatcatggccccggccttgatcgccaaccacagcgagctggatgagctggtggagaagacccggatagccgtagaccgcacggcgcggctggtcggcaagctgtaa

SEQ ID NO: 7 - DNA, 1362 bp, Aeromonas salmonicida subsp. salmonicida
  source 1..1362: mol_type = genomic DNA
atgcagcacacgacacgtgagtggcagcagctggatgccagccaccacctgcatccctttaccgattttcaggcgctgaaccagaagggcagccgcatcatcaccagggccgaaggcatctatctggaagactccgacgggcgtcgcattctggacggtatggcgggactctggtgcgtcaacatgggctacggtcgtcaggagctggtggaggctgccaccaaacagatgcagcaactgccctactacaaccttttcttccagaccgcacaccctcctgtgatcgagttggcgaccctgctggccgaggtgactccgtcccatctcaatcatgtcttcttcaccggttctggctccgagtgcaacgatacggtgctgcgcatggtccgccactactgggccagcaaggggcagccggacaagcaggtgatcatcagccgccacaacgcctatcacggctccaccgtggcgggtgccagtctgggtggcatgaagggcatgcacgcccagggcggcctgcccattcccggcatagtgcacatcgatcagccctatcacttcggtgaggggcagggaatgagtgcccacgagtttggtctggagcgtgcccgccagctggagcagaagatcctggagctgggggtggacaaggtggccgccttcatcggcgagcccatccagggcgccggcggcgtcatcattccgcccgacagctactggcccgagatccagcgcatctgtgacaagtacggcatcctgctcattgccgacgaggtgatctgcggctttggccgtaccggccactggttcgccagcgagggattcggcatcaagccggacctcatgtgcctggccaagggcatcacctcaggctatctgcccatgggggccgtgatggtgggggatcgcgttgccagggtgctggtggaggagggcggcgaattcaaccacggcttcacctattccggtcatccggtggcctgcgccgtcgccattgccaacattaagcttatgcaaagcgaaagcatagttaagcgaattcatgatactatcggcccctatttgcagcgccgctggcgcgaactggcagaccatccgctggtgggcgaaacccgtggcaaaggcctggtggccgcgctggaaatagtgcaggacaagcagaccaacagccgcttcccggctgggctgcaagccggcatgacctgccgggaattctgctttaacaatggcttggtgatgcgggcggtcggcgataccatgatcatatcgccccccttggtcatcaccgaggaacaggtggatgaattggtcaatctggccaggctcagtctggatctgacggctgcaaagctgaaagggtag

SEQ ID NO: 8 - DNA, 1380 bp, Escherichia coli K12 MG1655
  source 1..1380: mol_type = genomic DNA
ttgaacaggttaccttcgagcgcatcggctttagcgtgcagcgcccacgccctgaatctcattgagaagcgaacgctggatcatgaggagatgaaagcacttaaccgagaggtgattgaatacttcaaagagcatgtcaatccggggtttttagagtatcgcaaatctgttaccgccggcggggattacggagccgtagagtggcaagcgggaagtttaaatacgcttgtcgacacccagggccaggagtttatcgactgcctgggaggttttggaattttcaacgtggggcaccgtaatccagttgtggtttccgccgtacagaatcaacttgcgaaacaaccgctgcacagccaggagctgctcgatccgttacgggcgatgttggcgaaaacccttgctgcgctaacgcccggtaaactgaaatacagcttcttctgtaatagcggcaccgagtccgttgaagcagcgctgaagctggcgaaagcttaccagtcaccgcgcggcaagtttacttttattgccaccagcggcgcgttccacggtaaatcacttggcgcgctgtcggccacggcgaaatcgaccttccgcaaaccgtttatgccgttactgccgggcttccgtcatgtgccgtttggcaatatcgaagccatgcgcacggctcttaacgagtgcaaaaaaaccggtgatgatgtggctgcggtgatcctcgaaccgattcagggtgaaggtggcgtaattctgccgccgccgggctatctcaccgccgtacgtaagctatgcgatgagttcggcgcactgatgatcctcgatgaagtacaaacgggcatggggcgcacgggcaagatgttcgcctgcgagcatgagaacgtacagccggatatcctctgccttgccaaagcgctcggcggcggcgtgatgccgattggcgcgaccatcgccactgaagaggtgttttcagttctgttcgacaacccattcctgcataccaccacctttggcggcaacccgctggcctgtgcggcggcgctggcgaccatcaatgtgttgctggagcagaacttaccggctcaggctgagcaaaaaggcgatatgttgctggacggtttccgtcaactggcgcgggaatatcccgatctggtacaggaagcgcgtggtaaagggatgttgatggcgattgagtttgttgataacgaaatcggctataactttgccagcgagatgttccgccagcgcgtactggtggccggaacgctcaataacgccaaaacgatccgcattgaaccgccactgacactgaccattgaacagtgtgaactggtgatcaaagcggcgcgtaaggcgctggcggccatgcgagtaagtgtcgaagaagcgtaa

SEQ ID NO: 9 - DNA, 18 bp, synthetic construct
  source 1..18: mol_type = other DNA
ggatccgtgatggtgatg

SEQ ID NO: 10 - DNA, 20 bp, synthetic construct
  source 1..20: mol_type = other DNA
aagcttaattagctgagctt

SEQ ID NO: 11 - DNA, 33 bp, synthetic construct
  source 1..33: mol_type = other DNA
caccatcacggatccagcgtcaacaacccgcaa

SEQ ID NO: 12 - DNA, 34 bp, synthetic construct
  source 1..34: mol_type = other DNA
cagctaattaagcttttattgaatcgcctcaagg

SEQ ID NO: 13 - DNA, 31 bp, synthetic construct
  source 1..31: mol_type = other DNA
caccatcacggatccaacgcgcctttcgccc

SEQ ID NO: 14 - DNA, 33 bp, synthetic construct
  source 1..33: mol_type = other DNA
cagctaattaagcttttacagcttgccgaccag

SEQ ID NO: 15 - DNA, 32 bp, synthetic construct
  source 1..32: mol_type = other DNA
caccatcacggatcccagcacacgacacgtga

SEQ ID NO: 16 - DNA, 34 bp, synthetic construct
  source 1..34: mol_type = other DNA
cagctaattaagcttctaccctttcagctttgca

SEQ ID NO: 17 - DNA, 33 bp, synthetic construct
  source 1..33: mol_type = other DNA
caccatcacggatccaacaggttaccttcgagc

SEQ ID NO: 18 - DNA, 34 bp, synthetic construct
  source 1..34: mol_type = other DNA
cagctaattaagcttttacgcttcttcgacactt

SEQ ID NO: 19 - protein, 474 aa, Escherichia coli K12 MG1655
MQHKLLINGELVSGEGEKQPVYNPATGDVLLEIAEASAEQVDAAVRAADAAFAEWGQTTPKVRAECLLKLADVIEENGQVFAELESRNCGKPLHSAFNDEIPAIVDVFRFFAGAARCLNGLAAGEYLEGHTSMIRRDPLGVVASIAPWNYPLMMAAWKLAPALAAGNCVVLKPSEITPLTALKLAELAKDIFPAGVINILFGRGKTVGDPLTGHPKVRMVSLTGSIATGEHIISHTASSIKRTHMELGGKAPVIVFDDADIEAVVEGVRTFGYYNAGQDCTAACRIYAQKGIYDTLVEKLGAAVATLKSGAPDDESTELGPLSSLAHLERVGKAVEEAKATGHIKVITGGEKRKGNGYYYAPTLLAGALQDDAIVQKEVFGPVVSVTPFDNEEQVVNWANDSQYGLASSVWTKDVGRAHRVSARLQYGCTWVNTHFMLVSEMPHGGQKLSGYGKDMSLYGLEDYTVVRHVMVKH

SEQ ID NO: 20 - protein, 487 aa, Pseudomonas putida CSV86
MRETKEQPIWYGKVFSSNWVEARGGVANVVDPSNGDILGITGVANGEDVDAAVNAAKRAQKEWAAIPFSERAAIVRKAAEKLKEREHEFADWNVRECGAIRPKGLWEAGIAYEQMHQAAGLAYLSNGTLFPSAVPGRMNLCQRVPVGVVGVIAPWNFPLFLAMRSVAPALALGNAVILKPDLQTAVTGGALIAEIFSDAGMPDGVLHVLPGGADVGESMVANSGINMISFTGSTQVGRLIGEKCGRMLKKVALELGGNNVHIVLPDADLDGAVSCAAWGTFLHQGQVCMAAGRHLVHRDVAQQYAEKLALRAKNLVVGDPNSDRVHLGPLINDKQVVRVHALVESAQSAGAKVLAGGTYQDRYYQATVIMDVKPEMEVFKSEIFGPVAPITVFDSIEEAIELANCSEYGLAASIHTRALATGLDIAKRLNTGMVHINDQPINCEPHVPFGGMGASGSGGRFGGPASIEEFTQSQWISMVEKPANYPF

SEQ ID NO: 21 - protein, 496 aa, Pseudomonas putida S12
MNSSLSAIDGLRLPHQMLIGGQWVSAQSGKTLNVYNPATGDILTEVPDGDVEDVNAAVESAAATLRSDTWRRMPPSARERILLRLADLLEVHGDELARLETLNNGKLLIYSKLMEVGASAQWLRYMAGWATKLTGSTLDLSLPLPPEVRSRASTQRVPVGVVAAIIPWNFPLLMAVWKIAPALACGNTVVLKPAEETPLTALRLAELAMEAGLPAGALNVVTGRGETAGDALVRHPKVAKVAFTGSTEVGRIIGSACGRSLKAVSLELGGKSPVIVLADCDPQEAAEGAAAAIFFNHGQVCTAGSRLYVHESIYEDVIQRLAVIGESIVVGSGLEQGVHMGPMVSKKHHENVLRHIRNGIEDGADLICGGTEAPCAQGFFVKPTIFANREKKDIRLLSQEVFGPVLVATPFSDIAEVVNEANRSVYGLGASIWTNDLSAALRINDELEAGTVWVNTHNMVDPNLPFGGFKDSGVGREHGAAAIEHYTTTRSLVIAY

SEQ ID NO: 22 - protein, 491 aa, Pseudomonas putida NCIMB 9866
MSQRLAAYENMSLQLIAGEWRVGKAGRDLDVLDPFTQEKLLQIPLANREDLDEAYRSARQAQVAWAACGPSERAQVMLNAVRIFDERRDEIIDWIIRESGSTRIKAQIEWGAARAITQESASLPSRVHGRILASDVPGKESRVYREPLGVIGIISPWNFPLHLTARSLAPALALGNACVIKPASDTPVTGGLLLAHIFEEAGLPKGVLSVVVGSGSEIGDAFVEHEVPGFISFTGSTQVGRNIGRIAAGGEHLKHVALELGGNSPFVVLADADLDQAVNAAVVGKFLHQGQICMAINRIIVEDSVYDEFVNRYAERVKSLPYGDPSKPETVVGPVINAKQLAGLQDKIATAKSEGARVMVEGEAQGNVLPPHVFADVTADMEIAREEIFGPLVGIQRARDEAHALELANSSEYGLSSAVFTSSLERGVKFARGIRAGMTHINDIPVNDEPNAPFGGEKNSGLGRFNGDWAIEEFTTDHWITVQHAPRRYPF

SEQ ID NO: 23 - DNA, 1425 bp, Escherichia coli K12 MG1655
  source 1..1425: mol_type = genomic DNA
atgcaacataagttactgattaacggagaactggttagcggcgaaggggaaaaacagcctgtctataatccggcaacgggggacgttttactggaaattgccgaggcatccgcagagcaggtcgatgctgctgtgcgcgcggcagatgcagcatttgccgaatgggggcaaaccacgccgaaagtgcgtgcggaatgtctgctgaaactggctgatgttatcgaagaaaatggtcaggtttttgccgaactggagtcccgtaattgtggcaaaccgctgcatagtgcgttcaatgatgaaatcccggcgattgtcgatgtttttcgctttttcgcgggtgcggcgcgctgtctgaatggtctggcggcaggtgaatatcttgaaggtcatacttcgatgatccgtcgcgatccgttgggggtcgtggcttctatcgcaccgtggaattatccgctgatgatggccgcgtggaaacttgctccggcgctggcggcagggaactgcgtagtgcttaaaccatcagaaattaccccgctgaccgcgttgaagttggcagagctggcgaaagatatcttcccggcaggcgtgattaacatactgtttggcagaggcaaaacggtgggtgatccgctgaccggtcatcccaaagtgcggatggtgtcgctgacgggctctatcgccaccggcgagcacatcatcagccataccgcgtcgtccattaagcgtactcatatggaacttggtggcaaagcgccagtgattgtttttgatgatgcggatattgaagcagtggtcgaaggtgtacgtacatttggctattacaatgctggacaggattgtactgcggcttgtcggatctacgcgcaaaaaggcatttacgatacgctggtggaaaaactgggtgctgcggtggcaacgttaaaatctggtgcgccagatgacgagtctacggagcttggacctttaagctcgctggcgcatctcgaacgcgtcggcaaggcagtagaagaggcgaaagcgacagggcacatcaaagtgatcactggcggtgaaaagcgcaagggtaatggctattactatgcgccgacgctgctggctggcgcattacaggacgatgccatcgtgcaaaaagaggtatttggtccagtagtgagtgttacgcccttcgacaacgaagaacaggtggtgaactgggcgaatgacagccagtacggacttgcatcttcggtatggacgaaagatgtgggcagggcgcatcgcgtcagcgcacggctgcaatatggttgtacctgggtcaatacccatttcatgctggtaagtgaaatgccgcacggtgggcagaaactttctggttacggcaaggatatgtcactttatgggctggaggattacaccgtcgtccgccacgtcatggttaaacattaa

SEQ ID NO: 24 - DNA, 1464 bp, Pseudomonas putida CSV86
  source 1..1464: mol_type = genomic DNA
atgcgtgagaccaaggagcaaccgatctggtatggcaaggtgtttagcagcaactgggtggaggcgcgtggcggcgtggcgaatgtggttgatccgagcaacggtgacatcctgggtattaccggcgtggcgaacggtgaagatgtggatgcggcggttaacgcggcgaagcgtgcgcagaaagaatgggcggcgatcccgttcagcgagcgtgcggcgattgttcgtaaggcggcggaaaagctgaaagagcgtgaacacgagtttgcggattggaacgtgcgtgagtgcggtgcgatccgtccgaaaggcctgtgggaagcgggtattgcgtatgagcagatgcaccaagcggcgggcctggcgtatctgagcaacggtaccctgttcccgagcgcggttccgggtcgtatgaacctgtgccagcgtgtgccggttggtgtggttggcgtgatcgcgccgtggaacttcccgctgtttctggcgatgcgtagcgtggcgccggcgctggcgctgggtaacgcggttattctgaagccggatctgcaaaccgcggtgaccggtggcgcgctgattgcggaaattttcagcgatgcgggtatgccggatggtgtgctgcacgttctgccgggtggcgcggatgtgggtgaaagcatggttgcgaacagcggtatcaacatgattagctttaccggcagcacccaagttggtcgtctgatcggcgaaaaatgcggtcgtatgctgaagaaagtggcgctggagctgggtggcaacaacgtgcacattgttctgccggacgcggatctggatggtgcggttagctgcgcggcgtggggtaccttcctgcatcaaggtcaagtgtgcatggcggcgggtcgtcacctggtgcaccgtgatgttgcgcagcaatacgcggaaaagctggcgctgcgtgcgaaaaacctggtggttggtgatccgaacagcgaccgtgttcacctgggcccgctgatcaacgacaagcaggtggttcgtgtgcatgcgctggttgagagcgcgcaaagcgcgggtgcgaaagttctggcgggtggcacctaccaggatcgttactatcaagcgaccgtgattatggacgttaagccggaaatggaagtgttcaaaagcgaaatctttggtccggtggcgccgattaccgtttttgacagcatcgaggaagcgattgaactggcgaactgcagcgagtatggcctggcggcgagcattcatacccgtgcgctggcgaccggtctggatattgcgaagcgtctgaacaccggcatggttcacatcaacgaccagccgattaactgcgaaccgcatgttccgtttggtggcatgggtgcgagcggtagcggtggccgttttggtggcccggcgagcatcgaggaatttacccagagccagtggattagcatggtggagaaaccggcgaactacccgttttaa

SEQ ID NO: 25 - DNA, 1491 bp, Pseudomonas putida S12
  source 1..1491: mol_type = genomic DNA
atgaacagcagcctgagcgcgattgatggtctgcgtctgccgcaccagatgctgattggtggccagtgggttagcgcgcaaagcggcaagaccctgaacgtttacaacccggcgaccggcgacatcctgaccgaagtgccggacggtgatgtggaggatgttaacgcggcggttgaaagcgcggcggcgaccctgcgtagcgatacctggcgtcgtatgccgccaagcgcgcgtgaacgtatcctgctgcgtctggcggacctgctggaagtgcacggcgatgaactggcgcgtctggagaccctgaacaacggcaagctgctgatttacagcaaactgatggaagttggtgcgagcgcgcagtggctgcgttatatggcgggctgggcgaccaaactgaccggtagcaccctggacctgagcctgccgctgccgccggaagtgcgtagccgtgcgagcacccaacgtgtgccggttggtgtggttgcggcgatcattccgtggaacttcccgctgctgatggcggtttggaagattgcgccggcgctggcgtgcggtaacaccgtggttctgaaaccggcggaggaaaccccgctgaccgcgctgcgtctggcggagctggcgatggaagcgggtctgccggcgggtgcgctgaacgtggttaccggtcgtggcgagaccgcgggtgatgcgctggtgcgtcacccgaaggtggcgaaagttgcgtttaccggcagcaccgaagtgggtcgtatcattggtagcgcgtgcggtcgtagcctgaaggcggttagcctggagctgggtggcaaaagcccggtgatcgttctggcggactgcgacccgcaggaagcggcggagggtgcggcggcggcgattttctttaaccatggtcaagtgtgcaccgcgggtagccgtctgtacgttcacgagagcatctatgaagatgtgattcagcgtctggcggttatcggcgagagcattgtggttggtagcggcctggaacaaggcgtgcacatgggtccgatggttagcaagaaacaccacgagaacgttctgcgtcacatccgtaacggcattgaagacggtgcggatctgatctgcggtggcaccgaggcgccgtgcgcgcagggtttctttgtgaagccgaccatcttcgcgaaccgtgagaagaaagacattcgtctgctgagccaagaagttttcggcccggtgctggttgcgaccccgtttagcgatattgcggaagtggttaacgaagcgaaccgtagcgtgtatggtctgggcgcgagcatttggaccaacgacctgagcgcggcgctgcgtattaacgatgagctggaagcgggtaccgtgtgggttaacacccacaacatggtggacccgaacctgccgttcggtggctttaaagatagcggtgttggtcgtgagcatggtgcggcggcgatcgaacactacaccaccacccgtagcctggttattgcgtattaa

SEQ ID NO: 26 - DNA, 1476 bp, Pseudomonas putida NCIMB 9866
  source 1..1476: mol_type = genomic DNA
atgagccagcgtctggcggcgtacgagaacatgagcctgcaactgattgcgggtgaatggcgtgtgggcaaggcgggtcgtgacctggatgttctggacccgttcacccaggagaaactgctgcaaattccgctggcgaaccgtgaggacctggatgaagcgtatcgtagcgcgcgtcaggcgcaagttgcgtgggcggcgtgcggtccgagcgagcgtgcgcaggttatgctgaacgcggtgcgtatctttgatgagcgtcgtgacgaaatcattgattggatcattcgtgaaagcggcagcacccgtatcaaagcgcagattgagtggggtgcggcgcgtgcgatcacccaagaaagcgcgagcctgccgagccgtgttcatggtcgtattctggcgagcgatgttccgggcaaagagagccgtgtgtaccgtgaaccgctgggtgttatcggcatcattagcccgtggaacttcccgctgcacctgaccgcgcgtagcctggcgccggcgctggcgctgggcaacgcgtgcgtgattaaaccggcgagcgacaccccggttaccggtggcctgctgctggcgcacattttcgaggaagcgggtctgccgaaaggcgtgctgagcgtggttgtgggtagcggcagcgaaatcggtgatgcgtttgttgagcacgaagtgccgggtttcattagctttaccggcagcacccaagtgggtcgtaacattggtcgtattgcggcgggtggcgagcacctgaagcacgttgcgctggaactgggtggcaacagcccgttcgttgtgctggcggacgcggatctggaccaagcggtgaacgcggcggttgtgggtaaatttctgcaccagggccaaatctgcatggcgattaaccgtatcattgttgaggacagcgtgtacgatgaatttgtgaaccgttatgcggagcgtgttaagagcctgccgtatggtgacccgagcaaaccggaaaccgttgtgggcccggttatcaacgcgaagcagctggcgggtctgcaagataagattgcgaccgcgaaaagcgagggtgcgcgtgttatggtggaaggcgaggcgcagggtaacgtgctgccgccgcacgtttttgcggatgtgaccgcggatatggaaatcgcgcgtgaggaaatttttggtccgctggttggcattcagcgtgcgcgtgatgaggcgcatgcgctggaactggcgaacagcagcgagtacggcctgagcagcgcggtgttcaccagcagcctggaacgtggtgttaagtttgcgcgtggtattcgtgcgggcatgacccacatcaacgacattccggtgaacgatgagccgaacgcgccgttcggtggtgagaagaacagcggtctgggccgtttcaacggtgactgggcgatcgaggaatttaccaccgatcactggattaccgttcagcacgcgccgcgtcgttatccgttttaa

SEQ ID NO: 27 - DNA, 36 bp, synthetic construct
  source 1..36: mol_type = other DNA
caccatcacggatcccaacataagttactgattaac

SEQ ID NO: 28 - DNA, 36 bp, synthetic construct
  source 1..36: mol_type = other DNA
cagctaattaagcttttaatgtttaaccatgacgtg

SEQ ID NO: 29 - DNA, 34 bp, synthetic construct
  source 1..34: mol_type = other DNA
caccatcacggatcccgtgagaccaaggagcaac

SEQ ID NO: 30 - DNA, 35 bp, synthetic construct
  source 1..35: mol_type = other DNA
cagctaattaagcttttaaaacgggtagttcgccg

SEQ ID NO: 31 - DNA, 33 bp, synthetic construct
  source 1..33: mol_type = other DNA
caccatcacggatccaacagcagcctgagcgcg

SEQ ID NO: 32 - DNA, 37 bp, synthetic construct
  source 1..37: mol_type = other DNA
cagctaattaagcttttaatacgcaataaccaggcta

SEQ ID NO: 33 - DNA, 32 bp, synthetic construct
  source 1..32: mol_type = other DNA
caccatcacggatccagccagcgtctggcggc

SEQ ID NO: 34 - DNA, 35 bp, synthetic construct
  source 1..35: mol_type = other DNA
cagctaattaagcttttaaaacggataacgacgcg

SEQ ID NO: 35 - protein, 474 aa, Citrobacter koseri ATCC BAA-895
MPHQLLINGELVSGEGEKQPVYNPATGEVILEIAEASPAQVDAAVRAADRAFAEWGQTTPKARAELLLTLADVIEENAQTFAELESQNCGKPLHCALNDEIPAIVDVFRFFAGAARCLNGLAAGEYLEGHTSMIRRDPVGVVASIAPWNYPLMMAAWKLAPALAAGNCVVIKPSEITPLTALKLAEFAKDIFPPGVLNVLFGRGKTVGDPLTGHEKVRMVSLTGSIATGEHIIQHTAPSIKRTHMELGGKAPVIVFDDADLDAVVEGVRTFGFYNAGQDCTAACRIYAQKGIYDALVEKLGAAVASLKTGSPNDESTELGPLSSQAHLERVTKAVEEAKALGHINVVTGGQKLDGAGYYFAPTLLAGAKQEDAIVQREVFGPVVSMTVFDDEEQVLAWANDTQYGLASSVWTKDVGRAHRLSARLQYGCTWVNTHFMLVSEMPHGGQKRSGYGKDMSLYGLEDYTVIRHIMVKH

SEQ ID NO: 36 - protein, 474 aa, Salmonella enterica subsp. enterica serovar Choleraesuis str. SC-B67
MQYQLLINGVLVDGEGERQSVYNPATGEVILEIAEASPAQVDAAVLAADSAFAEWGQTTPKARAECLLKLADSIEQNALEFARLESQNCGKPLHCVINDEIPAIVDVFRFFAGAARCLSGLAAGEYLEGHTSMIRRDPIGVVASIAPWNYPLMMAAWKLAPALAAGNCVVIKPSEITPLTALKLAALAKDIFPPGVLNVLFGRGQTVGDVLTGHEKVRMVSLTGSIATGEHILRHTAPAIKRTHMELGGKAPVIVFDDADLDAAAQGVRTFGFYNAGQDCTAACRIYAQRGIYDALVEKLGNAVSSLKMGAPEDESTELGPLSSLAHLKRVTAAVEEAKALSHIRVITGGSQTEGKGYYFAPTLLADAKQEDAIVQREVFGPVVSITVFDDEDQVLRWANDSRYGLASSVWTQDVGRAHRLSARLQYGCTWINTHFMLVSEMPHGGQKQSGYGKDMSLYGLEDYTLVRHIMVKH

SEQ ID NO: 37 - protein, 474 aa, Pectobacterium atrosepticum SCRI1043
MHDKLLIEGKLIAGNGEALAVFNPATGEQIAAIPQADLHQIDAAVLAAESAFAHWGQTTPKTRATLLLKIADAIEENAEVFAKLESLNCGKPYHAVLNDEVPAVADVFRFFAGAARCLSGSAAGEYLEGHTSMIRRDPVGVVASIAPWNYPLMMASWKLAPALAAGNCVVLKPAEQTPLTTFYLAHLLADILPAGVVNIVFGRGADIGDALTGHEKVNMVSLTGSIATGAHILAHTAASVKRTHMELGGKAPVIVFDDADIDQVVDGIRSFGFYNAGQDCTAACRLYVQRAVYDEVVEALGKAVATLKIGDPRDETTELGPLITEPQLERVMGFVERAKALPHITVVTGGERVKGTGFYFQPTVLAGAKQDDEIVQKEVFGPVISITSFDDEAQVIGWANASNYGLASSVWTRDIGRAHRLAACLQYGCTWVNTHFMLVSEMPHGGQKLSGYGKDMSMYGLEDYTIVRHIMIRH

SEQ ID NO: 38 - protein, 474 aa, Cronobacter sakazakii ATCC 29544
MQSQLLINGALVEGKGERLPVYNPATGEVLLEIAEASPEQVDAAVKSADAAFEQWRLTTPKERAEALLKLADVIEANAQTFAQLESKNCGKPLHCVAGDEIPAVADVFRFFAGAARCLNGLAAGEYLADHTSMIRRDPVGVVASIAPWNYPLMMAAWKLAPALAAGNCVVLKPSEITPLTALKLAELAKDIFPAGVLNVLFGRGQTVGDPLTSHEKVRMVSLTGSIATGEHIISRTASSIKRTHMELGGKAPVLVFDDADLDAVVEGIRTFGFYNAGQDCTAACRIYAQKGMYDTLVEKLGTAVGSLKTGAPEDETTELGPLSSQAHLERVSQAVEAAKALPHIRVVTGGAKIDGPGYYFQPTVLAGAKQEDAIVQREVFGPVISVTPFEDEAQALTYANDSQYGLASSVWTRDVGRAHRLSARLQYGCTWVNTHFMLVSEMPHGGQKLSGYGKDMSMYGLEDYTVVRHVMIKH

SEQ ID NO: 39 - protein, 474 aa, Pseudomonas putida KT2440
MQTQMLINGQLVAGQGPAWTVLNPALGTALAQINEATEAQVDSAVRAADQAFDSWSQTSPKERSQALLALADAIEAHGDELARLESQNCGKPLSAALNDEIPAIADVFRFFAGAARCLGGSAAGEYLPGHTSMIRRDPLGVVASIAPWNYPLMMLAWKIAPALAAGNTVVIKPSELTPLTALRLGELAQDLLPPGVLNILFGRGQTVGNPLITHPKVRMVSLTGSIPTGAHIISATADSVKRMHMELGGKAPVLVFDDADIDAAIDGIRTFGFYNAGQDCTAACRLYVQDGIYERFVERLGKAVASLKPGLQESEETELGPLISAQHRDKVAGLVQRAIAQPHIRLVTGGKPIAGDGFFFEPTVLADALQDDEIVRNEVFGPVVSVTRFTDEAQALEWANDSNYGLASSVWTRDTGRAHRLAARLQYGCTWVNTHFMLVSEMPHGGQKHSGYGKDMSMYGLEDYTCVRHVMIKH

SEQ ID NO: 40 - protein, 488 aa, Halioxenophilus aromaticivorans
MQQERREASIWSGKVFSSGWVEARGGVCDVTDPSNGDLLGVTGIANGEDVAAAAQTARRAQKGWAAIPFSERAEIVRKAAEKLKERENEFADWNVRECGAIRQKGLWEAGITYQQMHQAASLAFLPDGTSFPSAVAGRLNLCQRVPVGVVGVIAPWNFPLFLSMRSVAPALVLGNAVVLKPDPQTAITGGALIAEIFSEAGLPDGVLHVLPGGAEAGESMVASPEIDMISFTGSTQVGRLIGEKCGGMLKKVALELGGNNVHIVLPDADLDGAASCAAWGTFLHQGQVCMAAGRHLVHRDIAQEYAEKLALRARNLVVGDPKTDQVHLGPLINDKQVAHVHALVESAQKAGAKILAGGAYQDRYYQATVLMDVTPKMDVFKLETFGPVAPITVVDSVEEAIELANSSEYGLAASIHTKSLATGLEIARNLKTGMVHINDQPINCEPHVPFGGMGASGSSGRFGGLASIDEFTQSQWISMVEKPSIYPF

SEQ ID NO: 41 - protein, 487 aa, Sphingomonas sp. TF3
MNTPIKSNAWTGKVFSHGWSAGSGGVAEVIEPATGEVLGQIGIADVKDVDAAVASARSAQEAWAATPFDQRAAIIRTAAEVLKRRAAEFVQWNTRECGSIPPKGEYEVGITYEQLQQAAALAALPNGSLFPSSVPGRTNLWQRVPLGVVGVIAPWNFPLFLAMRSVAPALSLGNAVVLKPDLQSAVTGGVLIAEIFEEAGLPDGVLHVLPGGAETGEALVRHPDVAMISFTGSTAVGRSIAEICGRMLKKVALELGGNNVHIVLPDADLDGAASCAAWGSFLHQGQVCMAAGRHLVHRSVVDEYAAKLATRAGALHVGDPNAGPCHLGPLINDRQVARVHEVVTGSIEAGAEVLTGGVHEGRFYQPTVLKGVTPEMSAFKSEIFGPVAPITVFDTEDEAIALSNRSEYGLAASIHTASAARGLALAKRLKTGMVHINDQPINCEPQVPFGGMGASGSGGRFGGPASIDEFTQAQWISLVEKPVIYPF

SEQ ID NO: 42 - protein, 487 aa, Rhodococcus imtechensis
MRRLLDEPVWESRIFTGEWVRGSADDHPVVEPATGKQLSTIGMATADDVTRAADRAATAQADWAARPYTERAAVLRRAGTLFEQHADEIAEWVIREAGSIPTKAHIETHTAAEECYNAAALAAHPYGEVLRSEQPRLSFSRRIPVGTVGVIAPFNFPIILSIRAVAPALALGNAVVLKPDPRTAICGGAVLARIFEEAGLPAGLLSVLPGGADAGEAVVVHRTVRVIAFTGSTRAGRAVGELAGRHLKRSHLELGGNNALIVLDDVDLEKAVAVGAFGSFMHQGQICMAAGRHLVHESIAADYTALLAEHADRLPVGDPFTGDVALGPIIDAKQRDHIHTLVTASIDAGATLAAGGTYDDLFYRPTVLAQTPLTAAAFQDEVFGPVAPVASFSSIEEAVTIANSSEYGLSLSILTADAMKGLELAQRIPAGLVHVNDQTVGDEAVVPFGGVGSSGNGGRVGGISANLDAFTETQWVTAQSTMPAYPF

SEQ ID NO: 43 - protein, 486 aa, Rhodococcus ruber
MALLDESIWQGKIFTGDWTPGGGGEIKVVEPATGATLGSAGLADEGDLERAVDRAVAAQGDWAARPHTERAAVMRRAGVLWQQHADEIERWIMRESGSLRPKAQLETHVAAQECYEGAALPSHALGEILPSEAPRLSMSKRVPVGVVGVIAPFNFPLILAIRSVAPALALGNAVILKPDPRTAVCGGVALARIFEQAGLPAGVLSVLPAGADVGAALVDDPRVPVISFTGSTPAGRAVGAAASRNLKKVHPELGGNSAIVVLDDADLAATVSAGAAGSFLHQGQVCMTTGRHIVHESVYDEYVAQLAAKAEALPVGDPVTEQVALGPIIDQGQLEKIHALVTASVDAGARLVAGGTYEGLFYRPTVLADVPAGAPAYAQEVFGPVAPVVKFSTLDEAVALATDTDYGLSLGIFTRDVGKGLALADRIPTGIAHINDQTVGDEANIPFGGLGASGNGARFGGAANSIEAFTESRWITVSRDVPAYPF

SEQ ID NO: 44 - protein, 496 aa, Pseudomonas sp. LQ26
MNSSLPNIDGLLSPNQMLIGGEWVNARSDKTLSVYNPATGEVLTEVPDADAADVDAAVEGASATLQSGVWRHMAPVARERILLRLADLLEAHGDELARLETLNNGKLLIYSKLMEVGASAQWLRYMAGWATKLTGNTLDLSLPLPPQVRTKASTQRLPIGVVAAIIPWNFPLLMAVWKITPALACGNTVVLKPAEETPLTALRLAELALEAGLPAGALNVVTGRGESAGDALVSHPKIAKVAFTGSTEVGRVIGAACGRSLKAVSLELGGKSPVIVLPDCDPQKAAEGAAAAIFFNHGQVCAAGSRLYVHESIYEDVIQRLAVIGQSIVLGSGLDQAAQMGPMVSQKHHENVLRHIRNGIEDGVDLVCGGADSPALPGYFVQPTVFANRQKKDIRLLSQEVFGPVLVATPFSDIQEVISEANRSVYGLGASIWTNDLSAALRINDELEAGTVWVNTHNMVDPNLPFGGFKDSGVGREHGAAAIEHYTTPRCHHIQC

SEQ ID NO: 45 - protein, 500 aa, Burkholderia lata
MYREISMPLEVTGSSLRTSMFINGEWQQANSGKMIPVFDPSNGERIASVPDADVADIDRAVESASLTFRSTSWKSMPPAARERILLRLADLIEKHGEELAALETRNNGKLIAYSRMFEVGAGTQWLRYMAGWATKISGSTLDLSLPLPPTVRTSAFTRRIPVGVVGAIIPWNFPLLMAVWKIAPALACGNTVVLKPAEETPLTALRLAELAVEAGLPAGALNVVTGRGETAGAALVAHPKVSKVTFTGSTEVGRLIGATCGQNLKPASLELGGKSPVIVLNDCDPDVAARGAADAIFFNHGQVCTAGSRLYVHHDIYDDVLDRLSAIADTIVVGSGFDESAHMGPLVSLRHQQRVKSLIESGRADGAEQLCGAGATPENGYYVRPTVFANHDNRPMRLLTEEVFGPVLVAMPFTDLAEVVDEANDSAYGLGASVWTNNLSASLALTEAIEAGTVWVNTHNMVDPNLPFGGFKDSGIGREHGASAIENYTTTKSVCIAYQG

SEQ ID NO: 46 - protein, 492 aa, Paraburkholderia sp. 5N
MTEQKTTAKLPTAMFINGEKTLSAAGKTFPIYNPATGQELSQIPDASETDIDHAVKTSKAAFESDTWRRMPPATRERLLLKLADLVEQHTDELATLETLNQGKLIVFSKMLEVTGSVQWLRYMAGWATKIEGTTFDLSVPFPPGTRYNASTKRVPAGVVAAIVPWNFPLLVAVWKIAPALACGCTVVLKPAEETPLTAIRLAELAHEAGFPPGVFNVVTGRGETAGAALVKHPLINKVTFTGSTEVGRIIGRQCADDLKRASLELGGKSPVIVLDDCDPKKAIEGAAGAIFFNHGQVCTAGSRLYVARSIYDEVVQGIAAVADGIALGSGFDAATQMGPMVSARHRDKVMGMIAQGRQEGGEILSRDAAVDAVGFFVRPTVIANRACKPLSVVREEVFGPVLVAMPYDDIDEVLAQANASEYGLGASVWTNQLDKALRLVDGIEAGTVWVNTHNMVDPAMPFGGFKASGIGREHGKAIVDSYTESKSVCIAY

SEQ ID NO: 47 - DNA, 1425 bp, Citrobacter koseri ATCC BAA-895
  source 1..1425: mol_type = genomic DNA
atgccgcatcagctgttgattaacggggaactggtatcaggggaaggagaaaagcaaccggtctataatccggcaaccggcgaagttatcctggaaattgcggaagcgagccccgcacaagtcgatgcagcggttcgtgcggcagatcgtgcgtttgccgaatggggccaaaccacaccgaaggcgcgtgcggaactcctccttacactggccgacgtcatcgaggaaaatgcccaaacgttcgccgaactcgagtcacagaattgcggtaaacccctgcattgcgccttgaatgacgaaattccagcgattgtggatgtgttccgcttctttgctggtgctgcccggtgtctgaatggtctggccgcaggggaatatctcgaaggtcatacatccatgattcgccgtgacccagtgggagtggttgcgtcgattgccccgtggaactatccgctgatgatggcggcttggaaactggctccagcgttagcagccggcaactgcgtcgttattaagccgtcagaaatcacgccactgacggcgctgaaactggcggagttcgccaaagacatctttcctcctggcgttttaaacgtgctgtttggtcgtggcaaaaccgtaggagatccgcttaccggccacgagaaagtgcgtatggtttcgcttacgggcagtatcgccactggcgaacacatcattcagcataccgccccgagcatcaaacgcacacatatggaactgggcggtaaagctcctgtcattgtgttcgatgatgcagatctggatgccgttgtagaaggtgtacggaccttcggcttttacaacgctggccaagattgcacggctgcatgtcgcatttacgcacagaaaggcatttatgacgccctggtagagaagctgggtgcggcggttgcaagcttgaaaaccggctctccgaacgatgagtccaccgagttgggtccgttaagcagtcaagcgcatctggagcgcgtgactaaagctgttgaagaagccaaagcgcttggccacatcaacgtcgtgactggtgggcagaaattggatggggcaggatactactttgcaccgactctgttagcgggcgcgaaacaggaggatgcgattgttcagcgcgaagtgtttggtcctgtggtcagtatgacggtctttgacgacgaggaacaggtgctggcttgggccaatgatacgcagtatgggttggcaagctctgtttggaccaaagacgtgggtcgcgctcatcgtctgtctgcgcgcttacagtacggctgtacctgggtaaacacccactttatgctggtgtccgaaatgccccatggaggtcagaaacgctcgggttatggtaaggacatgagcttatatggcctggaagattacaccgtgattcgccacatcatggtcaaacactaa

SEQ ID NO: 48 - DNA, 1425 bp, Salmonella enterica subsp. enterica serovar Choleraesuis str. SC-B67
  source 1..1425: mol_type = genomic DNA
atgcagtatcaactgctgattaatggcgtcttagtggacggcgaaggtgaacgccagtcagtctacaaccctgccaccggtgaggtaatcctggaaattgcggaagccagtccggcacaggtagatgcggctgttcttgcggcggatagtgcatttgcggaatggggtcaaaccaccccgaaagctcgtgcagaatgcctgctgaaactggcggatagcattgagcagaacgcactggaattcgcccgtttagagtcccaaaactgcggtaaacccttgcattgcgtgatcaacgacgaaattccggccatcgtagacgtctttcggttctttgcaggggctgcacgctgtctttctggtctggcggcgggcgaatacctggaaggccacacgagcatgattcgccgtgacccgattggagtcgtcgcgagtatcgcgccttggaactacccgctgatgatggccgcttggaaattggcaccagcactcgcggccggcaattgcgtagttatcaaaccgagcgaaattaccccgctgacggcgcttaaacttgccgcattggcaaaggatattttcccgccgggcgtcctgaatgtcttatttggccgtggtcagactgttggtgatgtgctgacaggtcacgaaaaggttcgcatggtgagtctgacaggttctattgccacaggagagcatattctgcgccatactgccccagcgatcaagcgtacgcacatggaactgggtggtaaagctcccgtgattgtgtttgacgatgctgatctggatgccgccgctcaaggcgttcgcacctttggcttttacaacgcgggacaagactgtacggctgcttgtcggatctatgcgcaacgtggcatctatgatgccctggtagaaaagttgggcaatgcggtgtcatccctgaaaatgggcgcgccggaagatgagtctacggaactcggaccactgtcctcattagcacatctcaaacgcgtgaccgcggccgttgaagaggccaaagctctgtcgcacattcgtgtaatcactggcgggagccagaccgaaggtaaagggtactatttcgccccaaccctcttagccgatgcgaaacaagaggatgcgattgtgcagcgtgaggtgtttggtcctgtcgtgtcgatcacggttttcgacgacgaggatcaggtgttacgttgggcgaatgattcgcgctatgggttggcgtccagcgtttggacccaggatgtgggtcgcgcacatcgcctgtcggcacgcttgcagtatgggtgtacctggatcaacacccacttcatgctggttagcgaaatgccgcatggcggccagaaacagtctggctatggcaaagacatgagcctttatgggctcgaagattacactctggttcgccacattatggtgaaacattaa

SEQ ID NO: 49 - DNA, 1425 bp, Pectobacterium atrosepticum SCRI1043
  source 1..1425: mol_type = genomic DNA
atgcacgacaaactgctgattgagggtaaactgatcgccggaaatggtgaagctctggcggtgtttaaccctgcgactggcgagcagattgcggcaattccacaggcagatcttcatcagattgatgcagccgtcttagcggctgaaagcgcctttgcccattggggccagacaaccccgaaaactcgcgctacgctgttacttaaaatcgcggacgccattgaggaaaatgccgaagtgtttgcgaaactggaatcgcttaactgcggcaaaccgtaccatgcagtgttgaacgacgaagttccagccgttgcggatgtgttccgcttctttgcgggagctgcccgttgtctgagcggctcagcggccggtgaatacttggaggggcatacctcgatgatccggcgtgatccggtgggagtagtggcgagcattgcgccgtggaactatccgctgatgatggctagctggaaactggcacccgccttagccgcgggtaattgcgtcgtgttgaaacccgcggaacaaacgccactcaccaccttttacctggcacatctgttagcggatattctgcctgctggtgtcgtaaacatcgttttcggtcgtggggctgatattggcgatgcattaaccgggcatgaaaaggtgaacatggtaagtctgaccgggtctattgccaccggcgcacatatcctggcacacacggccgcgtccgtaaaacgtacacacatggaactcggtggcaaagctccagtgattgtctttgatgatgccgacattgaccaagttgtcgacggcatccgctctttcggcttctataatgccggtcaagattgcaccgcggcatgtcgcctctacgtgcaacgcgcagtatatgatgaggtcgttgaagcgttgggtaaagcggttgcgaccctcaaaattggggatcctcgtgacgagacaacagaactgggtccgctgatcactgaaccgcaactggaacgcgtaatgggatttgtcgagcgtgctaaagccctgccgcacatcacggtcgtgactggaggtgaacgtgtgaagggcacggggttttacttccagccgactgttctggccggtgcgaaacaggatgacgaaatcgtgcagaaggaggttttcggcccggtgattagcattacgtcgtttgatgacgaagctcaggtcatcggttgggcaaatgcgagtaactatggcttggcgtcaagtgtgtggacccgcgatattggtcgcgcacatcggcttgcagcgtgcttacagtacggttgtacgtgggttaatacccactttatgctggtttccgaaatgccgcatggcggccagaagctgtctggctatggcaaagacatgtccatgtatggcctggaagattataccattgttcgccacatcatgatccgccactga

SEQ ID NO: 50 - DNA, 1425 bp, Cronobacter sakazakii ATCC 29544
  source 1..1425: mol_type = genomic DNA
atgcagagtcaattactgattaacggcgcgctggtggaaggcaagggcgagcgcctgccagtctataaccccgcgacgggcgaggtgctgctggagattgccgaagccagcccggaacaggtggatgcggcggtgaagagtgccgacgcggcgtttgaacagtggcgtctcaccacgcctaaagagcgcgccgaggcgctgctcaagcttgcagatgtgattgaggccaacgcgcagacctttgcgcagcttgaatctaaaaactgcggcaagccgctgcactgcgtggcgggtgacgaaatcccggcggtggcggatgtgttccgcttctttgccggcgccgcgcgctgcttaaacgggcttgccgccggggaatacctggcggatcacacctcgatgatccgccgtgacccggtgggcgtggtcgcgtccatcgcgccgtggaactacccgctgatgatggccgcctggaagctggcccccgcgctggcggcgggcaactgcgtggtgcttaagccctctgaaattacgccgctgaccgcgcttaagctcgcggagcttgccaaagatatcttcccggcgggtgtgcttaatgtgctgtttggccgtggccagacggtgggcgacccgctcaccagccatgagaaagtgcgcatggtgtcgctcaccggctctatcgccaccggcgagcacatcatcagccgcaccgcgtcgtccatcaagcgcacccatatggagcttggcggcaaagcgccggtgctggtgtttgacgacgccgatctcgacgccgtcgtcgaaggcatccgcacctttgggttctataacgcgggccaggactgtacggcggcgtgccgcatctacgcccaaaaagggatgtacgacacgctcgttgaaaaactcggcaccgcagtcggcagcctgaaaacaggcgcgccggaggatgaaaccaccgaactcgggccgctcagttcacaagcgcacctggagcgcgtgagccaggcggtggaggcggcgaaagcgctgccgcatattcgcgtggtgactggcggcgcgaaaatcgacgggccgggctattactttcagccgaccgttctcgccggcgcgaagcaggaggacgctatcgtgcagcgcgaggtgtttggcccggttatcagcgtgacgccgtttgaggatgaagcccaggcgctgacctacgccaacgattcgcaatatggcctggcgtcatccgtatggacccgcgacgtgggccgcgcgcaccgcctcagcgcccgcctgcaatatggctgcacctgggtgaatacgcacttcatgctggtgagcgaaatgccccacggcggccagaaactctccggctacggaaaggatatgtcgatgtacgggcttgaggattacaccgtcgtgcggcatgtaatgataaaacactag

SEQ ID NO: 51 - DNA, 1425 bp, Pseudomonas putida KT2440
  source 1..1425: mol_type = genomic DNA
atgcaaacgcagatgctgatcaatggccagctggtcgctggccaaggcccggcctggaccgtgctcaacccggcgctgggcactgccctggcgcagatcaacgaagccaccgaggcgcaggtggacagtgccgtgcgcgctgccgaccaggccttcgacagctggtcgcaaaccagccctaaagaacgttcgcaggccttgctggcgctggccgatgccatcgaagcccatggcgatgaactggcccggctggaatcacagaactgcggcaagcccctgagcgctgcactcaacgacgagatcccggcgattgccgacgtgttccgtttctttgccggtgcggcgcgctgcctgggcggctcggcggcaggcgagtacctgccgggccacacctcgatgatccgccgcgacccgttgggcgtggtggcttccatcgcgccgtggaactacccgctgatgatgctggcctggaagatcgccccagccctggctgccggcaacaccgtggtgataaagccgtccgagctgacgccgctgacggccctgcgcctgggcgagctggcccaggacttgctgccgccgggggtgctgaacattctcttcggccgcggccagacggtcggcaacccgttgataacccaccccaaggtgcgcatggtgtcgctgaccggctcgatccccaccggcgcgcacatcatcagcgccaccgccgacagcgtgaaacgcatgcacatggagctgggcggcaaggcgccggtgctggtgttcgatgacgctgacatcgatgccgccatcgacggcatccgcaccttcggcttctacaacgccggccaggactgcaccgcagcctgccgcctgtatgtgcaggacgggatctacgagcgctttgtcgaacgcctgggtaaagccgtagccagcctcaagccgggcctgcaggagtctgaagaaaccgaactggggccactgatcagcgcccagcaccgcgacaaggtcgccgggctggtgcagcgggccatcgcccagccgcacattcgtctggtaaccggtggcaagccaatagcgggcgatggctttttcttcgagcctaccgtgctggccgacgccctgcaggacgacgagatcgtgcgcaacgaagtgtttggcccggtggtttcggtcacccgcttcaccgatgaagcgcaggcactggaatgggccaacgactccaactacggcctggcctcatcggtatggacccgcgacaccggccgcgcccaccgcctggcggcgcgcttgcagtatggctgcacctgggtgaatacccacttcatgctggtcagcgaaatgccccatggcgggcagaagcattcggggtatggcaaggacatgtcgatgtatgggctggaggactacacctgtgtgcggcatgtgatgatcaagcattga

SEQ ID NO: 52 - DNA, 1467 bp, Halioxenophilus aromaticivorans
  source 1..1467: mol_type = genomic DNA
atgcaacaggagcgtcgcgaagcatcgatttggagtggtaaagtgtttagctccggttgggtggaggcacgtggcggagtttgcgacgtgaccgatccaagcaatggcgatctgcttggtgtcacagggattgccaatggtgaggacgtcgcagcggcagcacagacagcccgtcgcgctcagaaaggctgggctgcgatcccgttctccgaacgtgctgaaatcgtgcgtaaagcagccgagaagctcaaagaacgcgagaacgaattcgccgattggaatgtccgcgaatgtggtgccattcgccagaaagggctgtgggaagctggcatcacctatcagcagatgcatcaagcggctagtctggcgtttctgccggatggcacctcctttccgtcagcggttgccggtcgcttaaacctgtgtcaacgtgtgcctgtaggagtggtcggagtgattgctccgtggaactttccgctgttccttagcatgcgttctgtggcgccagcgttggttctcgggaatgccgtagtactgaaaccggatccacagacggccattacgggcggagccttgatcgcggagatcttctctgaagcaggcttaccggatggtgtcttacacgttctgccgggtggtgcagaagcgggcgaaagcatggttgcttcgccagagatcgacatgatctcatttactggcagcactcaggtcggccgcctgatcggcgagaaatgcggcggcatgctgaagaaagtggctttagaacttggtgggaataacgtgcacattgtgcttcctgacgcagatttggatggcgcggcgtcttgtgcggcctggggtacgttcctgcatcaggggcaagtatgcatggcggcaggccgtcacctggtgcatcgcgacattgcacaggagtatgcggagaagctggccttacgggctcgcaatctggttgttggggatccgaaaacggatcaagtccatctcggtcctctgatcaacgacaaacaagtagcgcatgttcatgcgctggtagaatcggcccagaaagcgggagcaaagattctggccggcggtgcgtaccaggatcgctactatcaggctaccgttctcatggatgttacgccgaaaatggacgtgttcaaactggaaacatttggccccgtggcccctattaccgtcgtagattcggtcgaagaagcgatcgaattggcgaacagttcggaatatggcctggcggcgagcatccacaccaaatctttggccactggtctggaaattgcccgcaatctgaaaaccggcatggtgcacattaacgatcaaccgattaactgcgaaccccatgttccgtttggcgggatgggtgccagtggtagttccgggcggttcggtggcctggcatcaattgacgaatttacccagagccaatggatttcaatggtggaaaagcccagcatttacccgttttga

SEQ ID NO: 53 - DNA, 1464 bp, Sphingomonas sp. TF3
  source 1..1464: mol_type = genomic DNA
atgaacaccccgatcaagtcaaacgcttggactggtaaagtgttttcccacggctggtctgcaggcagcggtggggtagccgaagtgatcgagccggcaaccggagaagtactggggcagattgggattgcggatgtcaaagatgttgatgcggccgtcgctagcgctcgttcggcgcaggaagcgtgggctgctacccctttcgaccagcgtgccgccatcattcggacagctgcagaagtccttaaacgccgtgctgcggaatttgttcagtggaatacgcgcgaatgcggttccattccgccgaaaggggagtatgaggtggggattacctacgaacagctgcaacaggcggctgctcttgccgcgttgccaaacggatcgctgtttccctcatccgtgcctggacgtaccaatctgtggcagcgcgtgccactcggagtcgttggcgttatcgcaccttggaactttccgttgttcctcgcgatgcgtagcgtggcgcctgcattatcgttgggcaatgccgtggtgttaaaaccggatctccaatcagcagttacaggtggcgttctgattgcggaaattttcgaagaagccgggcttccggatggcgttttgcacgtgttacccggcggggccgaaacgggtgaagcgctggtgcgccatcccgacgtagcgatgatttcctttacgggtagtaccgcggttggccgtagcattgccgagatttgtggccgcatgctgaagaaagttgctctggagctgggtggcaataacgtgcacattgtcctgccggatgcggatctcgatggcgcagcgagttgtgcggcgtggggttcattcctgcatcaaggccaagtctgcatggccgcaggccgtcatcttgtgcatcgcagcgtcgtggacgagtatgcggcgaaactggcaacccgcgccggtgccttacatgtaggggacccaaatgccggtccttgtcacctgggtccgctgatcaacgatcgccaagtagcgcgcgttcatgaggtagttacgggatcgatcgaagcgggtgcagaagtgctgacgggcggtgtgcatgaaggccgcttttaccagccaactgtgctgaaaggcgtcacaccggaaatgtcggcgttcaaaagcgaaatcttcggcccggttgcaccgattactgtctttgatacggaagatgaggctattgccctgagtaaccgcagcgaatatggcttagcagcatctattcacaccgcgtctgcggcacgcggtctggccctggccaagcggttgaaaactggtatggtgcacatcaacgaccaaccgatcaattgcgaaccacaggtaccgtttggtggcatgggagcctctggcagtggcggtcgtttcggtggccccgccagcatcgacgaatttacccaggcacagtggatcagtctggtggagaaaccggtcatttacccgttttaa

SEQ ID NO: 54 - DNA, 1464 bp, Rhodococcus imtechensis
  source 1..1464: mol_type = genomic DNA
gtgcggcggttgctggacgaaccggtgtgggaatcacgaatcttcaccggcgaatgggtacgcggcagcgccgacgaccaccccgttgtcgagcccgcaaccggcaaacaactctcgaccatcggcatggccaccgcagacgatgtgacacgtgccgcggaccgagccgcgaccgcgcaagccgactgggccgcccgcccctacaccgaacgggcagcagtgctccgccgcgccggaaccctgttcgagcagcacgccgacgaaatcgccgaatgggtgatccgcgaggccggcagcatccccaccaaggcccacatcgaaacacacaccgccgccgaggagtgctacaacgctgcggcgcttgccgcacacccctacggtgaagtgctgcgctcggagcagccgcgcttgagcttctcccgccgcatcccggtgggcaccgtcggggtgatcgcccccttcaacttcccgatcatcctgtcgatccgtgccgtcgcgccggcgttggcgctcggtaacgccgtcgtcctcaagcccgacccccgcaccgccatctgtggcggtgcggtcctcgcccgcatcttcgaggaagccggccttcccgccggcctgctcagcgtgctgcccggcggcgccgacgccggggaagccgtcgtcgtccaccgcaccgttcgggtcatcgccttcaccggttcgacccgcgccgggcgtgccgtcggtgaactcgccggacggcacctcaaacgctcccacctcgaactcggtggcaacaacgccctgatcgtgctcgacgacgtcgacctcgagaaggccgtagccgtcggcgctttcggctccttcatgcaccagggccagatctgcatggcggcgggccgtcacctggtgcacgagagcatcgccgccgactacaccgcactcctcgctgaacacgccgaccggctgcccgtcggtgacccgttcaccggcgacgtcgccctcggcccgatcatcgatgccaaacaacgagatcacatccacaccctggtcaccgcgagcatcgatgcgggcgccaccctcgcggccggcggaacctacgacgatctcttctaccggcccaccgtgctcgcgcagaccccgctgaccgccgcggccttccaggacgaggttttcggcccggtagccccggtggcatcgttcagttcgatcgaggaagccgtgacgatcgccaacagctccgaatacgggctgtcgttgagcatcctgacagccgacgccatgaagggcctcgaactcgcacagcggatccccgccggcctggtgcacgtcaacgaccaaaccgtgggcgacgaggcagtagtcccgttcggcggcgtcggatcctcgggcaacggcgggcgggtcggcggcatcagcgccaacctcgacgccttcaccgaaacacagtgggtcaccgcgcaaagcacgatgcccgcttacccgttctga

SEQ ID NO: 55 - DNA, 1461 bp, Rhodococcus ruber
  source 1..1461: mol_type = genomic DNA
atggcccttctcgacgaatccatctggcagggaaaaatcttcaccggggactggacccccggcgggggcggtgagatcaaggtcgtcgaaccggcgaccggcgcgacgctcggcagcgccggcctcgccgacgagggggacctcgagcgcgcggtcgaccgtgccgtcgcggcccagggcgactgggcggcccgcccgcacaccgagcgtgccgcggtcatgcgccgggccggcgtcctgtggcagcagcacgccgacgagatcgagcgctggatcatgcgcgagtccggctccctgcgtcccaaggcgcagctcgagacgcacgtcgcggcgcaggagtgctacgagggtgcggccctgccctcccatgcgctcggcgagatcctgcccagcgaggcaccgcgtctgagcatgtcgaagcgggtccccgtcggggtcgtcggtgtcatcgcgccgttcaacttcccgttgatcctcgcgatccgttccgtcgcgccggcgctggccctcggcaacgccgtgatcctcaagcccgacccgcgtaccgcggtctgcggcggcgtggcgctcgcccgcatcttcgagcaggcgggcctgccggccggggtgctgtccgtgctgcccgccggcgccgacgtcggcgccgcgctcgtcgacgacccgcgggtgccggtgatctccttcaccggttccaccccggccggccgggccgtcggtgccgccgcctcccgcaacctcaagaaggtccaccccgaactcggcggcaactccgcgatcgtcgtgctcgacgacgccgacctcgccgccaccgtctcggccggtgccgccggatccttcctgcaccagggccaggtgtgcatgaccaccggccggcacatcgtgcacgagtccgtctacgacgagtacgtcgcccagctcgccgccaaggccgaggcactgcccgtcggcgaccccgtcaccgagcaggtcgcgctcgggccgatcatcgaccagggtcagctcgagaagattcatgccctggtcaccgcgtcggtcgatgccggcgcccggctcgtcgccggcggcacctacgagggcctgttctaccggcccaccgtcctcgccgacgtcccggccggtgcgcccgcctacgcccaagaggtgttcgggcccgtcgctccggtcgtgaagttctcgaccctcgacgaggcggtggcgctggccaccgacaccgactacgggctctcgctcggcatcttcacccgcgacgtcggcaagggtctcgcgctcgcggaccggatccccaccggcatcgcccacatcaacgaccagaccgtcggcgacgaggccaacatcccgttcggcggtctcggcgcctccggcaacggcgcccgcttcggcggtgccgccaacagcatcgaagcgttcaccgagtcgcgctggatcaccgtcagccgcgacgtgcccgcttaccccttctga

SEQ ID NO: 56 - DNA, 1491 bp, Pseudomonas sp. LQ26
  source 1..1491: mol_type = genomic DNA
atgaacagctcacttccgaacattgacggtctgcttagccctaaccagatgctgattggtggcgaatgggtaaatgcccgctcggacaaaaccttgtccgtgtataatccggcaactggtgaagtgctgaccgaggttccggatgcggatgcggcagacgtagacgcggccgtggaaggcgctagtgccaccctccagtctggtgtgtggcgtcatatggctccagtggcacgtgaacgcatcctgctgcgcttagcggatctgctggaagcgcatggggatgaactggctcgcttggaaaccctcaacaatgggaaacttctcatctattcgaaactgatggaagtgggcgcaagcgcccaatggctgcgctatatggcggggtgggcgaccaagctgacgggtaacactctggacctgtcattaccgctgccgccgcaagtgcgtaccaaagcctctacgcagcgtctgcccattggagttgtagcagccatcattccctggaactttccgctgttaatggccgtttggaaaatcaccccagcgttagcttgcggcaataccgtcgtgctgaaaccggcggaggaaaccccgctgacagcgctccggttggcggaacttgcgctggaagcaggcttgcctgctggtgcactgaacgtggtaactggacgcggtgaaagcgccggggatgcgttagtcagccatccgaaaattgccaaagtggcttttaccggaagtaccgaagttggccgggttattggggcggcatgtggtcgctctctgaaagcggtaagcctggaactgggcggcaaaagtccggtaatcgtccttcccgactgtgatccgcagaaagcggcagagggcgcagctgccgcgatcttcttcaaccacggtcaagtttgcgccgcaggatctcgtctgtatgtccatgagtcgatttacgaggatgtcatccaacgcctggctgtgattggccagtccatcgtcttggggtccggcctcgatcaagccgcccagatgggcccaatggtatcgcagaaacaccacgagaacgttttacgccatattcgcaatggcattgaagatggcgtggatctggtttgtggtggcgcggatagcccggcacttccaggttactttgtgcaacctacggtgtttgcgaatcgccagaagaaggacattcgcctgctcagtcaggaggttttcggtcccgttttagtcgctacaccgtttagcgatattcaggaggtgatctcggaagcaaatcgttcagtctatggcttgggcgcgagtatctggacgaatgatctgtcagccgccctgcgtatcaacgacgaactggaagccggaactgtctgggttaatacgcacaacatggtcgacccgaacttgccatttggcgggttcaaggattccggtgtgggtcgtgagcatggtgcggcggctattgaacactacacaacgcctcgttgccatcacattcagtgctga

SEQ ID NO: 57 - DNA, 1503 bp, Burkholderia lata
  source 1..1503: mol_type = genomic DNA
atgtatcgcgaaatttctatgccgctggaagtaaccggttcttctctgcgtaccagcatgttcatcaacggtgaatggcaacaggccaattccggcaagatgattccggtgtttgatccgtcaaacggtgagcgtatcgcctccgttccggatgcggacgtagcggacattgatcgcgccgttgagagtgcttcgctcactttccgcagtacctcgtggaaaagcatgcctccagcagcgcgcgaacgcattttactgcgtctggcagatctgatcgagaaacatggcgaagagctggccgcacttgaaacgcgcaacaacggcaagttgattgcgtatagtcggatgttcgaggttggcgctggtacccaatggctgcgctatatggcagggtgggcgactaagatttccggtagcaccctggatctctctctccctctgccgccaacagtgcgtactagtgcatttactcgccgcattcccgtgggtgtggtgggtgcgattatcccgtggaactttccgctgctgatggctgtctggaaaatcgccccagcgttagcgtgcggtaataccgtagttctgaaaccagccgaagaaaccccgctgactgccttacgtttagccgaattggcggttgaggccggattgcctgcgggcgcactgaatgtagtcacaggccgtggcgaaaccgcaggagcagcactggttgcccatccgaaagtcagcaaagtgacctttaccggcagcacagaagttggtcgtcttattggggcgacgtgtggtcagaaccttaaaccagcgagcttggaacttggagggaaatctccggtgattgtcctgaacgactgcgacccggatgtcgcagctcgtggtgctgcagatgctatcttcttcaatcatggccaggtgtgtactgcggggtcccgtctgtacgttcatcacgacatctacgatgatgtgcttgaccgcctgagcgcgattgccgatacgatcgttgtcggcagcggctttgacgaatcagcgcacatgggtccgctggtgtcgctccgtcatcagcaacgcgtcaaaagcttaatcgaatcaggccgcgctgatggagcagaacagctgtgtggtgctggcgccacgcccgaaaacgggtactatgttcgcccgaccgtgtttgcgaatcacgataatcggcccatgcggctgctgaccgaggaagtatttggccccgtgttggtagcaatgccgtttaccgatctggctgaagtggtggacgaagccaatgacagcgcgtatggcctcggcgcgagtgtctggacgaacaacttatcggcgtcattggccctgacggaggccattgaagctgggaccgtgtgggtcaacacgcacaatatggttgatcctaatctgccgtttggcggcttcaaagattccgggattggacgcgaacatggtgcctcggcgattgagaactatacgacgacaaaatcggtgtgcatcgcgtaccagggttga

SEQ ID NO: 58 - DNA, 1479 bp, Paraburkholderia sp. 5N
  source 1..1479: mol_type = genomic DNA
atgacagaacagaaaaccaccgcgaaactgccgactgctatgtttatcaacggcgagaaaaccctgagtgcagcgggcaagacgtttcccatctacaatcctgcgacaggtcaggaattgtcacagatcccagacgcgtcggaaaccgatattgaccatgcggtaaagaccagtaaagccgcgtttgagagtgacacttggcgccgcatgccgccggccacccgtgagcgtctgctgctgaaactcgcggacttggttgagcagcatacggacgaactggcaaccttagaaactctgaaccagggtaagctcattgtgttttccaaaatgctggaggtcactggctcagtccagtggttgcggtatatggccggttgggcaaccaaaatcgaggggacgacctttgatctgtccgtaccgtttcctccaggcacacgctacaacgcgagcaccaaacgcgttcctgccggcgttgtggcggccattgtgccatggaactttccgttattggttgctgtgtggaaaattgccccggcgttagcgtgtggctgtaccgtcgtgcttaaaccggcggaagagactccgcttaccgcaattcgtctggctgaactggctcatgaagctgggtttccgcccggggtattcaacgttgtcacaggacgtggtgaaaccgcaggggctgcactggtcaaacacccgctgattaacaaggtgacgttcacgggtagcaccgaagttggtcgcatcattggccgccaatgcgcggatgaccttaaacgcgcatctctggaactcggtggtaaatcgccggtaattgtcctggatgattgcgatccgaagaaagccattgaaggcgctgccggagcaatcttcttcaatcacggtcaagtgtgtactgccggttcgcgcctgtatgtggcccgcagcatctacgacgaagtggtgcagggtattgcagccgttgcagatgggattgccctgggcagtggttttgatgcggccacgcaaatgggccccatggtgtcagcacgtcatcgtgacaaagtgatgggcatgattgcacagggtcgccaagaaggcggagaaatcctttctcgggatgctgccgttgatgctgtggggttcttcgtgcgcccaacggtgatcgccaatcgtgcgtgcaaaccgttgagcgtagttcgcgaagaagtctttggccctgttctggtagcgatgccctatgatgacattgatgaagtgttagcgcaagcaaatgcttcggagtatggcctgggtgcgtctgtctggacgaatcagttagataaggccctccgtctggtggatggtattgaagcgggcacagtctgggttaacacgcacaatatggtcgatccagccatgccgttcggcggattcaaagcgagcggcattggacgtgaacatggcaaagcgatcgttgattcctacaccgagagcaaaagcgtatgcatcgcgtattga

SEQ ID NO: 59 - DNA, 36 bp, synthetic construct
  source 1..36: mol_type = other DNA
caccatcacggatccatgccgcatcagctgttgatt

SEQ ID NO: 60 - DNA, 37 bp, synthetic construct
  source 1..37: mol_type = other DNA
cagctaattaagcttttagtgtttgaccatgatgtgg

SEQ ID NO: 61 - DNA, 38 bp, synthetic construct
  source 1..38: mol_type = other DNA
caccatcacggatccatgcagtatcaactgctgattaa

SEQ ID NO: 62 - DNA, 38 bp, synthetic construct
  source 1..38: mol_type = other DNA
cagctaattaagcttttaatgtttcaccataatgtggc

SEQ ID NO: 63 - DNA, 37 bp, synthetic construct
  source 1..37: mol_type = other DNA
caccatcacggatccatgcacgacaaactgctgattg

SEQ ID NO: 64 - DNA, 36 bp, synthetic construct
  source 1..36: mol_type = other DNA
cagctaattaagctttcagtggcggatcatgatgtg

SEQ ID NO: 65 - DNA, 37 bp, synthetic construct
  source 1..37: mol_type = other DNA
caccatcacggatcccagagtcaattactgattaacg

SEQ ID NO: 66 - DNA, 38 bp, synthetic construct
  source 1..38: mol_type = other DNA
cagctaattaagcttctagtgttttatcattacatgcc

SEQ ID NO: 67 - DNA, 37 bp, synthetic construct
  source 1..37: mol_type = other DNA
caccatcacggatcccaaacgcagatgctgatcaatg

SEQ ID NO: 68 - DNA, 37 bp, synthetic construct
  source 1..37: mol_type = other DNA
cagctaattaagctttcaatgcttgatcatcacatgc

SEQ ID NO: 69 - DNA, 34 bp, synthetic construct
  source 1..34: mol_type = other DNA
caccatcacggatcccaacaggagcgtcgcgaag

SEQ ID NO: 70 - DNA, 36 bp, synthetic construct
  source 1..36: mol_type = other DNA
cagctaattaagctttcaaaacgggtaaatgctggg

SEQ ID NO: 71 - DNA, 36 bp, synthetic construct
  source 1..36: mol_type = other DNA
caccatcacggatccaacaccccgatcaagtcaaac

SEQ ID NO: 72 - DNA, 36 bp, synthetic construct
  source 1..36: mol_type = other DNA
cagctaattaagcttttaaaacgggtaaatgaccgg

SEQ ID NO: 73 - DNA, 34 bp, synthetic construct
  source 1..34: mol_type = other DNA
caccatcacggatcccggcggttgctggacgaac

SEQ ID NO: 74 - DNA, 34 bp, synthetic construct
  source 1..34: mol_type = other DNA
cagctaattaagctttcagaacgggtaagcgggc

SEQ ID NO: 75 - DNA, 35 bp, synthetic construct
  source 1..35: mol_type = other DNA
caccatcacggatccgcccttctcgacgaatccat

SEQ ID NO: 76 - DNA, 34 bp, synthetic construct
  source 1..34: mol_type = other DNA
cagctaattaagctttcagaaggggtaagcgggc

SEQ ID NO: 77 - DNA, 36 bp, synthetic construct
  source 1..36: mol_type = other DNA
caccatcacggatccatgaacagctcacttccgaac

SEQ ID NO: 78 - DNA, 35 bp, synthetic construct
  source 1..35: mol_type = other DNA
cagctaattaagctttcagcactgaatgtgatggc

SEQ ID NO: 79 - DNA, 37 bp, synthetic construct
  source 1..37: mol_type = other DNA
caccatcacggatccatgtatcgcgaaatttctatgc

SEQ ID NO: 80 - DNA, 34 bp, synthetic construct
  source 1..34: mol_type = other DNA
cagctaattaagctttcaaccctggtacgcgatg

SEQ ID NO: 81 - DNA, 36 bp, synthetic construct
  source 1..36: mol_type = other DNA
caccatcacggatccatgacagaacagaaaaccacc

SEQ ID NO: 82 - DNA, 35 bp, synthetic construct
  source 1..35: mol_type = other DNA
cagctaattaagctttcaatacgcgatgcatacgc

SEQ ID NO: 83 - DNA, 36 bp, synthetic construct
  source 1..36: mol_type = other DNA
caccatcacggatccatcataggggttcctaaagag

SEQ ID NO: 84 - DNA, 35 bp, synthetic construct
  source 1..35: mol_type = other DNA
cagctaattaagcttttaagcacccgccacagatg

SEQ ID NO: 85 - DNA, 39 bp, synthetic construct
  source 1..39: mol_type = other DNA
caccatcacggatccacgaatactctggatgttttaaaa

SEQ ID NO: 86 - DNA, 38 bp, synthetic construct
  source 1..38: mol_type = other DNA
cagctaattaagcttttacagccaagttgatacttttg

SEQ ID NO: 87 - DNA, 23 bp, synthetic construct
  source 1..23: mol_type = other DNA
catggtatatctccttcttaaag

SEQ ID NO: 88 - DNA, 18 bp, synthetic construct
  source 1..18: mol_type = other DNA
ctcgagcaccaccaccac

SEQ ID NO: 89 - DNA, 40 bp, synthetic construct
  source 1..40: mol_type = other DNA
taagaaggagatataccatgaacaggttaccttcgagcgc

SEQ ID NO: 90 - DNA, 41 bp, synthetic construct
  source 1..41: mol_type = other DNA
catggtatatctccttcttattacgcttcttcgacacttac

SEQ ID NO: 91 - DNA, 39 bp, synthetic construct
  source 1..39: mol_type = other DNA
taagaaggagatataccatgcgtgagaccaaggagcaac

SEQ ID NO: 92 - DNA, 40 bp, synthetic construct
  source 1..40: mol_type = other DNA
tggtggtggtggtgctcgagttaaaacgggtagttcgccg

SEQ ID NO: 93 - DNA, 39 bp, synthetic construct; identical to SEQ ID NO: 91
  source 1..39: mol_type = other DNA

SEQ ID NO: 94 - DNA, 40 bp, synthetic construct
  source 1..40: mol_type = other DNA
catggtatatctccttcttattaaaacgggtagttcgccg

SEQ ID NO: 95 - DNA, 40 bp, synthetic construct; identical to SEQ ID NO: 89
  source 1..40: mol_type = other DNA

SEQ ID NO: 96 - DNA, 41 bp, synthetic construct
  source 1..41: mol_type = other DNA
tggtggtggtggtgctcgagttacgcttcttcgacacttac

SEQ ID NO: 97 - DNA, 21 bp, synthetic construct
  source 1..21: mol_type = other DNA
catagctgtttcctgtgtgaa

SEQ ID NO: 98 - DNA, 20 bp, synthetic construct
  source 1..20: mol_type = other DNA
gaattcactggccgtcgttt

SEQ ID NO: 99 - DNA, 40 bp, synthetic construct
  source 1..40: mol_type = other DNA
tcacacaggaaacagctatgaacaggttaccttcgagcgc

SEQ ID NO: 100 - DNA, 40 bp, synthetic construct
  source 1..40: mol_type = other DNA
aaacgacggccagtgaattcttaaaacgggtagttcgccg

SEQ ID NO: 101 - DNA, 39 bp, synthetic construct
  source 1..39: mol_type = other DNA
tcacacaggaaacagctatgcgtgagaccaaggagcaac

SEQ ID NO: 102 - DNA, 41 bp, synthetic construct
  source 1..41: mol_type = other DNA
aaacgacggccagtgaattcttacgcttcttcgacacttac

SEQ ID NO: 103 - protein, 454 aa, Pseudomonas chlororaphis subsp. aureofaciens NBRC 3521
MTSNNPQTREWQTLSSEHHLAPFSDFKQLKEKGPRIITNAEGVYLWDSEGNKILDGMAGLWCVAIGYGREELADAASKQMRELPYYNLFFQTAHPPALELAKAISDVAPQGMNHVFFTGSGSEGNDTMLRMVRHYWAIKGQPKKKTIISRVNGYHGSTVAGASLGGMTYMHEQGDLPIPGIVHIPQPYWFGEGGDMTPDEFGIWAANQLEEKILELGVDNVGAFIAEPIQGAGGVIVPPESYWPRIKEILAKYDILFVADEVICGFGRTGEWFGSDFYDLKPDMMTIAKGLTSGYIPMGGLIVRDEVVAVLNEGGDFNHGFTYSGHPVAAAVALENIRIMRDEKIIERVKAETAPYLQKRLRELNDHPLVGEVRGVGLLGAIELVQDKATRARYVGKGVGMICRQFCFDNGLIMRAVGDTMIIAPPLVITKEEIDELVSKARKCLDLTLSALQG

SEQ ID NO: 104 - protein, 456 aa, Pseudomonas aeruginosa PAO1
MNSQITNAKTREWQALSRDHHLPPFTDYKQLNEKGARIITKAEGVYIWDSEGNKILDAMAGLWCVNVGYGREELVQAATRQMRELPFYNLFFQTAHPPVVELAKAIADVAPEGMNHVFFTGSGSEANDTVLRMVRHYWATKGQPQKKVVIGRWNGYHGSTVAGVSLGGMKALHEQGDFPIPGIVHIAQPYWYGEGGDMSPDEFGVWAAEQLEKKILEVGEENVAAFIAEPIQGAGGVIVPPDTYWPKIREILAKYDILFIADEVICGFGRTGEWFGSQYYGNAPDLMPIAKGLTSGYIPMGGVVVRDEIVEVLNQGGEFYHGFTYSGHPVAAAVALENIRILREEKIIEKVKAETAPYLQKRWQELADHPLVGEARGVGMVAALELVKNKKTRERFTDKGVGMLCREHCFRNGLIMRAVGDTMIISPPLVIDPSQIDELITLARKCLDQTAAAVLA

SEQ ID NO: 105 - protein, 462 aa, Halomonas elongata DSM 2581
GMQTQDYQALDRAHHLHPFTDFKALGEEGSRVVTHAEGVYIHDSEGNRILDGMAGLWCVNLGYGRRELVEAATAQLEQLPYYNTFFKTTHPPAVRLAEKLCDLAPAHINRVFFTGSGSEANDTVLRMVRRYWALKGQPDKQWIIGRENAYHGSTLAGMSLGGMAPMHAQGGPCVPGIAHIRQPYWFGEGRDMSPEAFGQTCAEALEEKILELGEEKVAAFIAEPVQGAGGAIMPPESYWPAVKKVLAKYDILLVADEVICGFGRLGEWFGSQHYGLEPDLMPIAKGLSSGYLPIGGVLVGDRVAETLIEEGGEFFHGFTYSGHPTCAAVALKNLELLEAEGVVDRVRDDLGPYLAERWASLVDHPIVGEARSLGLMGALELVADKTTGQRFDKSLGAGNLCRDLCFANGLVMRSVGDTMIISPPLVIRREEIDELVELARRALDETARQLTQVPHTQEEPTA

SEQ ID NO: 106 - protein, 469 aa, Halomonas elongata DSM 2581
MTTHKDLIDRDRKVTFHASTHLRDFAHGDAPGRVITGGKGIKIVDKDGREFIDGFAGLYCVNIGYGRSEVAEAIYQQALEMSYYHTYVGHSNEPQIALSEKILELAGPGMSKVYYGMSGSDANETQLKIVRYYNNVLGRPQKKKVISRMRGYHGSGIASGSLTGLKAFHDHFDLPIETIRHTEAPYYYHRAAEQEGMTEREFSKHCAAKLEEMILAEGPDTVAAFIGEPVLGTGGIVPPPEGYWDEIQAVLTKYDVLLIADEVVCGFGRTGSDFGSHHYGIKPDLITIAKGLTSAYQPLSGVIVGDRVWEVLEQGTGEYGPIGHGWTYSGHALGCAAGLANLAIIEREGLTANAAETGAYLQERMKAAFADHPVVGQVRGVGMMAALEFSVDPAARRHFDPSLKVGPRMSAAALEEDLIARAMPQGDILGFAPPLTTTREEVDEIVARTERAVNKVTDALTREGAIQAA

SEQ ID NO: 107 - protein, 395 aa, Methanosarcina acetivorans C2A
METRTLEDWRALLEAEKTLDSGVYNKHDLLIVRGQGARVWDAEGNEYIDCVGGYGVANLGHGNPEVVEAVKRQAETLMAMPQTLPTPMRGEFYRTLTAILPPELNRVFPVNSGTEANEAALKFARAHTGRKKFVAAMRGFSGRTMGSLSVTWEPKYREPFLPLVEPVEFIPYNDVEALKRAVDEETAAVILEPVQGEGGVRPATPEFLRAAREITQEKGALLILDEIQTGMGRTGKRFAFEHFGIVPDILTLAKALGGGVPLGVAVMREEVARSMPKGGHGTTFGGNPLAMAAGVAAIRYLERTRLWERAAELGPWFMEKLRAIPSPKIREVRGMGLMVGLELKEKAAPYIARLEKEHRVLALQAGPTVIRFLPPLVIEKEDLERVVEAVRAVLA

SEQ ID NO: 108 - DNA, 1365 bp, Pseudomonas chlororaphis subsp. aureofaciens NBRC 3521
  source 1..1365: mol_type = genomic DNA
atgaccagcaacaacccgcaaacccgtgagtggcaaaccctcagcagcgagcaccacctggcacccttcagcgacttcaagcagttgaaggagaaggggccgcggatcatcactaatgccgagggcgtttacctctgggacagcgagggcaacaagatcctcgacggtatggccgggctgtggtgcgtggccatcggttacggccgcgaagaactggccgacgccgccagcaagcagatgcgcgagctgccgtactacaacctgttcttccagaccgcccacccgccggcgctggaactggccaaggccatctccgatgttgctccgcagggcatgaaccatgtgttcttcaccggttccggctccgaaggcaacgacaccatgctgcgcatggttcgccactactgggcgatcaagggccagccgaagaagaaaaccatcatcagccgggtcaacggctatcacggttccaccgtggccggcgcgagcctgggcggcatgacctatatgcacgaacagggcgacttgccgatcccaggcatcgtgcatatcccgcagccttactggttcggtgaaggcggcgacatgaccccggacgagttcgggatctgggcggccaaccagctggaagagaagattctcgaactcggcgtcgacaacgtcggtgccttcattgccgagccgatccagggcgcgggcggcgtgatcgtgccgccggaaagctactggccgcggatcaaggagatccttgccaagtacgacatcctgttcgtcgccgacgaggtgatctgtgggttcgggcgtaccggtgagtggttcggtagcgatttctacgacctcaagccggacatgatgactatcgccaagggcctgacttccggctacatccccatgggtggcctgatcgtgcgcgacgaagtggtggcggtgctcaacgagggcggcgatttcaaccacggtttcacctattccgggcacccggtggccgccgccgtggccctggaaaacatccgcatcatgcgcgacgagaaaattatcgagcgcgtcaaggcagaaacggcaccttatttgcagaaacgtctgcgggaactgaacgatcacccgctggtgggtgaggttcgcggagtcggcctgttgggcgccatcgaactggttcaggacaaggccacccgtgcgcggtatgtcggaaaaggcgtcggcatgatctgccggcagttctgcttcgacaacggcctgatcatgcgcgccgtgggcgacaccatgatcattgctccgcccctggtgatcaccaaggaggagatcgatgagctggtgagcaaggcccgcaagtgcctggacctgaccttgagtgcgttgcagggctaa

SEQ ID NO: 109 - DNA, 1371 bp, Pseudomonas aeruginosa PAO1
  source 1..1371: mol_type = genomic DNA
atgaacagccaaatcaccaacgccaagacccgtgagtggcaggcgttgagccgcgaccaccatctgccgccgttcaccgactacaagcagttgaacgagaagggcgcgcggatcatcaccaaggccgaaggcgtctatatctgggacagcgagggcaacaagatcctcgatgcgatggccggcctctggtgcgtcaacgtcggctacggccgcgaggagctggtccaggccgccacccggcagatgcgcgagttgccgttctacaacctgttcttccagaccgcccacccgccggtggtcgagctggccaaggcgatcgccgacgtcgctccggaaggcatgaaccacgtgttcttcaccggctccggctccgaggccaacgacaccgtgctgcgtatggtccgccactattgggcgaccaagggccagccgcagaagaaagtggtgatcggccgctggaacggctaccacggctccaccgtcgccggcgtcagcctgggcggcatgaaggcgttgcatgagcagggtgatttccccatcccgggcatcgtccacatcgcccagccctactggtacggcgagggcggcgacatgtcgccggacgagttcggcgtctgggccgccgagcagttggagaagaagattctcgaagtgggcgaggaaaacgtcgccgccttcatcgccgagccgatccagggcgccggcggcgtgatcgtcccgccggacacctactggccgaagatccgcgagatcctcgccaagtacgacatcctgttcatcgccgacgaagtgatctgcggcttcggccgtaccggcgagtggttcggcagccagtactacggcaacgccccggacctgatgccgatcgccaagggcctcacctccggctacatccccatgggcggggtggtggtgcgcgacgagatcgtcgaagtgctcaaccagggcggcgagttctaccacggcttcacctattccggtcacccggtggcggccgccgtggccctggagaacatccgcatcctgcgcgaagagaagatcatcgagaaggtgaaggcggaaacggcaccgtatttgcagaaacgctggcaggagctggccgaccacccgttggtgggcgaagcgcgcggggtcggcatggtcgccgccctggagctggtcaagaacaagaagacccgcgagcgtttcaccgacaagggcgtcgggatgctgtgccgggaacattgtttccgcaacggtttgatcatgcgcgcggtgggcgacactatgattatctcgccgccgctggtgatcgatccgtcgcagatcgatgagttgatcaccctggcgcgcaagtgcctcgatcagaccgccgccgccgtcctggcttga

SEQ ID NO: 110 - DNA, 1386 bp, Halomonas elongata DSM 2581
  source 1..1386: mol_type = genomic DNA
atgcaaacccaagactatcaggccctggaccgcgcccatcacctgcatcccttcaccgatttcaaggcgttgggtgaagagggcagtcgcgtcgtgacccacgccgaaggcgtctacatccacgacagcgagggcaaccgcattctcgacggcatggccgggctttggtgcgtgaatctcggctatggtcgccgcgaactggtcgaggcggcaacggcgcagctcgagcaactgccgtactacaacaccttcttcaagaccacgcatccgcccgcggtgcgcctggccgagaagctgtgcgatctagcgccggcgcacatcaatcgtgtgttcttcaccggctccggttccgaggccaacgacaccgtgctgcgcatggtacggcgttactgggccttgaagggccaacccgacaagcaatggatcatcggtcgcgagaacgcctatcacggctccaccctggccggcatgagcctgggcggcatggcgccgatgcatgcccagggcggcccctgcgtgcccggcatcgcccacatccgccagccctactggttcggcgaggggcgggacatgtcgccggaggccttcggccagacgtgcgctgaggcgctggaggagaaaatcctcgagctcggcgaggagaaggtggccgctttcatcgccgaaccggtgcagggcgccgggggggccatcatgccgccggagagctactggccggccgtcaagaaagtgctggcgaaatacgacatcctgctggtcgccgacgaggtgatctgcggcttcgggcgactcggcgagtggttcggcagccagcactacggtctcgagcccgacctgatgccgatcgccaagggcctgtcctccggctatctaccgatcggcggcgtgctggtcggggatcgtgtcgccgagacgctgatcgaagaaggcggcgagttcttccacggtttcacctactcggggcatccgacctgtgccgccgtggcgctcaaaaacctcgagctactcgaggccgagggcgtggtggatcgggtgcgcgacgatcttggtccctatctggccgagcgctgggccagcctggtcgaccatcctatcgtcggcgaggcacgatccctgggcctgatgggtgccctggaactggtcgccgacaagaccaccgggcagcgtttcgacaagtcgctgggcgccggcaacctgtgccgtgacctgtgcttcgccaatggcctggtgatgcgctccgtgggcgataccatgatcatttcgccaccgctggtgattcgtcgcgaggaaatcgacgaactggtggaactggcccgacgggccctggacgagacggctcgccaactgacgcaagtgccgcacacgcaagaggagccaaccgcatga

SEQ ID NO: 111 - DNA, 1410 bp, Halomonas elongata DSM 2581
  source 1..1410: mol_type = genomic DNA
atgaccactcacaaggatctgatcgatcgcgaccgcaaggtgaccttccacgcctccacccacctgcgcgacttcgcccatggcgacgcgccgggccgggtgatcaccggcggcaagggcatcaagatcgtcgacaaggacggccgcgagttcatcgacggcttcgccggcctgtattgcgtcaacatcggctacggccgcagcgaggtcgccgaggcgatttatcagcaggccctggagatgtcctactaccatacctatgtgggccactccaacgagccgcagatcgcgctttccgagaagatcctcgagctggccggccccggcatgtccaaggtctactacggcatgtccggcagcgacgccaatgagacccagctcaagatcgtgcgttactacaacaacgtgctcggccgcccgcagaagaagaaagtcatctcgcgcatgcgcggctatcacggctccggcatcgcctccggctcgctgaccgggctgaaggcgttccacgatcatttcgacctgccgatcgagacgatccgccacaccgaggcgccgtactactatcatcgtgccgccgagcaggaaggcatgaccgagcgcgagttctccaagcattgtgccgccaagctggaggagatgatcctggccgaaggaccggacaccgtggctgccttcatcggcgagccggtgctcggcaccggcggcatcgtgccgccgcccgaaggctactgggacgagatccaggcggtgctgaccaagtacgacgtgctgctgatcgccgacgaagtggtgtgcggcttcggtcgcacgggcagcgacttcggcagccatcactacggcatcaagccggacctgatcaccatcgccaagggcctgaccagcgcctatcagccgctctccggggtgatcgttggcgaccgcgtctgggaagtgctcgagcagggcaccggcgaatacggcccgatcggccacggctggacctattccggccacgccctgggctgtgccgccgggctggccaacctggcgatcatcgaacgcgaaggcctcaccgccaacgccgccgagaccggcgcctacctgcaggagcgcatgaaggctgccttcgccgaccatccggtcgtcggccaggtgcgtggcgtgggcatgatggcggcgctggagttttccgtcgacccggcggcgcgtcgtcacttcgatccgtccctcaaggtcgggccgcgcatgtccgccgccgccctcgaggaagacctgatcgcacgcgccatgccgcagggcgatatcctcggcttcgcgccgccgctgaccaccactcgcgaggaagtcgacgagatcgtcgcgcgcaccgagcgggcggtgaacaaggtgaccgatgcgctgacgcgggaaggtgccatccaggccgcctga

SEQ ID NO: 112 - DNA, 1188 bp, Methanosarcina acetivorans C2
  source 1..1188: mol_type = genomic DNA
gtggaaacgagaaccctggaagactggcgggcccttttggaggcggagaagaccctggacagcggcgtctacaacaagcacgacctcctcatcgtccggggccagggcgcgagggtctgggacgcggaaggcaacgagtacattgactgcgtgggcgggtacggggtggccaacctgggccacggcaaccccgaggtggtggaggcggtgaagcggcaggcggagacccttatggccatgccccagaccctccccacccccatgcggggggagttctaccgcaccctcaccgccatcctccccccggagctcaaccgggtcttccccgtgaactcgggcaccgaggccaacgaggccgccctaaagttcgcccgggcccacacgggcaggaagaagttcgtggccgccatgcggggcttctccgggcgaaccatgggaagcctctccgtcacctgggagcccaagtaccgggagcctttcttgcccttggtggagcccgtggagttcatcccctacaacgacgtggaggccctcaagcgggccgtggacgaggagacggccgcggtgatcctggagcccgtgcaaggggaggggggcgtgcgcccggcgacccccgagttcctaagggccgcccgggagatcacccaggagaagggggccctcctcatcctggacgagatccagaccggaatgggccgcacggggaagcgcttcgcctttgagcacttcggcatcgtccccgacatcctcaccctggccaaggccctcgggggcggggtgcccctgggggccgcggtgatgcgggaggaggtggcgcggagcatgcccaagggggggcacggcaccaccttcggggggaatcccctggccatggccgcaggggtggcggccatccgctacctggagcggacgcggctttgggaaagggccgcggagcttgggccctggttcatggagaagcttagggccatcccctcccccaagatccgggaggtgcggggcatgggcctcatggtgggcctggagctcaaggaaaaggccgccccctacatcgccaggctggagaaggagcaccgcgtcctcgccctccaggctgggcccacggtgatccgcttcctgccgcctttggtcattgaaaaggaagacctggagcgggtggtggaggcggtgcgggcggtgctagcatag

SEQ ID NO: 113 - DNA, 35 bp, synthetic construct
  source 1..35: mol_type = other DNA
caccatcacggatccaccagcaacaacccgcaaac

SEQ ID NO: 114 - DNA, 34 bp, synthetic construct
  source 1..34: mol_type = other DNA
cagctaattaagcttttagccctgcaacgcactc

SEQ ID NO: 115 - DNA, 35 bp, synthetic construct
  source 1..35: mol_type = other DNA
caccatcacggatccaacagccaaatcaccaacgc

SEQ ID NO: 116 - DNA, 33 bp, synthetic construct
  source 1..33: mol_type = other DNA
cagctaattaagctttcaagccaggacggcggc

SEQ ID NO: 117 - DNA, 35 bp, synthetic construct
  source 1..35: mol_type = other DNA
caccatcacggatcccaaacccaagactatcaggc

SEQ ID NO: 118 - DNA, 35 bp, synthetic construct
  source 1..35: mol_type = other DNA
cagctaattaagctttcatgcggttggctcctctt

SEQ ID NO: 119 - DNA, 36 bp, synthetic construct
  source 1..36: mol_type = other DNA
caccatcacggatccaccactcacaaggatctgatc

SEQ ID NO: 120 - DNA, 33 bp, synthetic construct
  source 1..33: mol_type = other DNA
cagctaattaagctttcaggcggcctggatggc

SEQ ID NO: 121 - DNA, 39 bp, synthetic construct
  source 1..39: mol_type = other DNA
caccatcacggatccatcacaaattcaaggaaaggaatt

SEQ ID NO: 122 - DNA, 36 bp, synthetic construct
  source 1..36: mol_type = other DNA
cagctaattaagctttcaggcctgctcaagaacatc

SEQ ID NO: 123 - protein, 378 aa, Bacillus subtilis 168
MIIGVPKEIKNNENRVALTPGGVSQLISNGHRVLVETGAGLGSGFENEAYESAGAEIIADPKQVWDAEMVMKVKEPLPEEYVYFRKGLVLFTYLHLAAEPELAQALKDKGVTAIAYETVSEGRTLPLLTPMSEVAGRMAAQIGAQFLEKPKGGKGILLAGVPGVSRGKVTIIGGGVVGTNAAKMAVGLGADVTIIDLNADRLRQLDDIFGHQIKTLISNPVNIADAVAEADLLICAVLIPGAKAPTLVTEEMVKQMKPGSVIVDVAIDQGGIVETVDHITTHDQPTYEKHGVVHYAVANMPGAVPRTSTIALTNVTVPYALQIANKGAVKALADNTALRAGLNTANGHVTYEAVARDLGYEYVPAEKALQDESSVAGA

SEQ ID NO: 124 - DNA, 1137 bp, Bacillus subtilis 168
  source 1..1137: mol_type = genomic DNA
atgatcataggggttcctaaagagataaaaaacaatgaaaaccgtgtcgcattaacacccgggggcgtttctcagctcatttcaaacggccaccgggtgctggttgaaacaggcgcgggccttggaagcggatttgaaaatgaagcctatgagtcagcaggagcggaaatcattgctgatccgaagcaggtctgggacgccgaaatggtcatgaaagtaaaagaaccgctgccggaagaatatgtttattttcgcaaaggacttgtgctgtttacgtaccttcatttagcagctgagcctgagcttgcacaggccttgaaggataaaggagtaactgccatcgcatatgaaacggtcagtgaaggccggacattgcctcttctgacgccaatgtcagaggttgcgggcagaatggcagcgcaaatcggcgctcaattcttagaaaagcctaaaggcggaaaaggcattctgcttgccggggtgcctggcgtttcccgcggaaaagtaacaattatcggaggaggcgttgtcgggacaaacgcggcgaaaatggctgtcggcctcggtgcagatgtgacgatcattgacttaaacgcagaccgcttgcgccagcttgatgacatcttcggccatcagattaaaacgttaatttctaatccggtcaatattgctgatgctgtggcggaagcggatctcctcatttgcgcggtattaattccgggtgctaaagctccgactcttgtcactgaggaaatggtaaaacaaatgaaacccggttcagttattgttgatgtagcgatcgaccaaggcggcatcgtcgaaactgtcgaccatatcacaacacatgatcagccaacatatgaaaaacacggggttgtgcattatgctgtagcgaacatgccaggcgcagtccctcgtacatcaacaatcgccctgactaacgttactgttccatacgcgctgcaaatcgcgaacaaaggggcagtaaaagcgctcgcagacaatacggcactgagagcgggtttaaacaccgcaaacggacacgtgacctatgaagctgtagcaagagatctaggctatgagtatgttcctgccgagaaagctttacaggatgaatcatctgtggcgggtgcttaa

SEQ ID NO: 125 - protein, 202 aa, Bacillus subtilis 168
MTNTLDVLKARASVKEYDTNAPISKEELTELLDLATKAPSAWNLQHWHFTVFHSDESKAELLPVAYNQKQIVESSAVVAILGDLKANENGEEVYAELASQGYITDEIKQTLLGQINGAYQSEQFARDSAFLNASLAAMQLMIAAKAKGYDTCAIGGFNKEQFQKQFDISERYVPVMLISIGKAVKPAHQSNRLPLSKVSTWL

SEQ ID NO: 126 - DNA, 609 bp, Bacillus subtilis 168
  source 1..609: mol_type = genomic DNA
atgacgaatactctggatgttttaaaagcacgtgcatctgtaaaggaatatgatacaaatgccccgatctctaaggaggagctgactgagctattagaccttgccactaaagcgccttctgcttggaaccttcagcattggcattttacagtattccacagcgatgaatcaaaagcggagcttcttcctgtagcgtataatcaaaaacaaatcgttgagtcttctgctgttgttgccattttaggcgatttaaaggcaaatgaaaacggtgaagaagtttatgctgaattagcaagccaaggctatattacggatgaaatcaaacaaacattgctcggccaaatcaacggtgcttaccaaagcgagcaattcgcacgtgattccgctttcttaaatgcttctttagctgctatgcagcttatgattgccgcaaaagcaaaaggttatgacacttgcgcaatcggcggatttaacaaagagcagttccaaaagcaatttgatatcagtgagcgctatgttccggttatgcttatttcaatcggcaaagcagtgaagcctgcgcatcaaagcaaccgtctgccgctttcaaaagtatcaacttggctgtaa

SEQ ID NO: 127 - protein, 487 aa, Hydrogenophaga aromaticivorans
MNTPVKTERWSGKIFTGSWVAARGGVAPVLEAATGAALGEVGVASPEDVDAAARSAQAAQKAWAATPFDQRAAIVREAARLLKERAAEFTQWNVRECGSIVPKGEWEVGITHEQMQQAAALAGLPNGMMFPSSVPGRTNLWQRVPLGVVGVIAPWNFPLFLAMRSVAPALALGNAVLLKPDLQSAVTGGALIARLFEDVGLPPGVLQVLPGGPATGDAVVRHPCVNMVSFTGSTAVGRQIGEFCGRALKKVALELGGNNAMIVLDDADLDGASSCAAWGGFLHQGQICMAAGRHLVHRSVADAYAAKLVERAKKLYVGDPHAGPAHLGPLINDRQTERVHRIVTESIAAGATLLAGGTHEGRFYQPTVLSNVAVDMPAFAEEIFGPVAPITVFDTDEEAVALANSSEYGLAAAIHSKSTARALRMASQLKSGMVHINDQPVNCEPQVPFGGMGASGSGGRFGGPASIDEFTQAQWVSVSEKAAQYPF

SEQ ID NO: 128 - protein, 487 aa, Pseudomonas aeruginosa
MRETKEQPIWYGKVFSSNWVEARGGVANVVDPSNGDILGITGVANGEDVDAAVNAAKRAQKEWAAIPFSERAAIVRKAAEKLKEREHEFADWNVRECGAIRPKGLWEAGIAYEQMHQAAGLAYLSNGTLFPSAVPGRMNLCQRVPVGVVGVIAPWNFPLFLAMRSVAPALALGNAVILKPDLQTAVTGGALIAEIFSDAGMPDGVLHVLPGGADVGESMVANSGINMISFTGSTQVGRLIGEKCGRMLKKVALELGGNNVHIVLPDADLDGAVSCAAWGTFLHQGQVCMAAGRHLVHRDVAQQYAEKLALRAKNLVVGDPNSDRVHLGPLINDKQVVRVHALVESAQSAGAKVLAGGTYQDRYYQATVIMDVKPEMEVFKSEIFGPVAPITVFDSIEEAIELANCSEYGLAASIHTRALATGLDIAKRLNTGMVHINDQPINCEPHVPFGGMGSSGSGGRFGGLASIDEFTQSQWISMVEKSASYPF

SEQ ID NO: 129 - protein, 487 aa, Pseudomonas sp. MAP12
MHETKEQPIWGGKIFSSTWVEARGGVANVVDPSNGDILGITGVANREDVDVAVSAAKIAQKEWAAMPFSERAAIVRKAADKLKEREHEFADWNVRECGAIRPKGLWEAGITYEQMHQAVGLASLPNGALFPSAVSGRMNLCQRVPIGVVGVIAPWNFPLFLAMRSVAPALVLGNAVVLKADLQTAVIGGALIAEIFSDAGIPEGVLHVLPGGADVGESMVENPGINMISFTGSTQVGRSIGEKCGRMLKKVSLELGGNNVNIVLPDADLDGAVGCAAWGTFFHQGQVCMAAGRHLVHRDIAQEYAAKLAKRAQSLVVGDPNTDQVHLGPLINDKQVDRVHALVESAERAGAKVLAGGAYEGRYYQATVVMDVKPDMEIFQSEIFGPVAPITIFDSIDEAIELANSSEYGLAASIHTKSLTTGMKIANRLKTGMVHINDQPINCEPHVPFGGMGASGSGGRFGGTASIEEFTQSQWISVVDKTAVYPF

SEQ ID NO: 130 - protein, 489 aa, Alteromonas
MQQERKKEVPIWSGKVFSSGWVEARGGASDVTDPSNGDLLGVVGIANGEDVAAAAQSARRAQKEWAAIPFSERAEIVRKAAEKLKERENEFADWNVRECGAIRQKGLWEAGITYQQMHQAASLAFLPDGTSLPSTVAGRLNLCHRVPVGVVGVIAPWNFPLFLAMRSVAPALVLGNAVILKPDPQTAVTGGALIAEIFSEAGIPDGVIHVLPGGAEAGESMVTNPGIDMISFTGSTEVGRLIGEKCGRMLKKVALELGGNNVHIILPDADLDGAASCAAWGTFLHQGQVCMAAGRHLVHRDIAQEYAEKLALRARNLVVGDPKTDQVHLGPLVNDKQVAHVHALVESAQKAGAKILAGGTYQDRYYQATVLMDVTPKMDIFELETFGPVAPITIVDSVEEAIGLANSSEYGLAASIHTKDLAAGLEIARNLKTGMVHINDQPINCEPHVPFGGMGASGSSGRFGGLASIDAFTQSQWISMVGKPATYPF

SEQ ID NO: 131 - protein, 487 aa, Tepidiphilus succinatimandens
MNWNGKLPIWHGKVFSNGWVVPRGGVADVVDPSSGDVLGVTGIANSEDIATAASAAKEAQKKWAAMPFNDRAAILRKAAEKLREREAEFADWNVRECGAVRMKGVWEAGITYEQMHQAASLAFLPNGTLFPSQVPGRMNFVHRVPVGVVGVIAPWNFPLFLAMRSVAPALVLGNAVILKPDVQTAVTGGALIAEIFAEAGIPEGVLHVLPGGADAGDAMVTNPEIDMISFTGSTAVGRQIGEKCGRMLKKVTLELGGNNVHIVLPDADLTGAASCAAWGTFLHQGQVCMAAGRHLVHRDVAQQYAQELAARAKNLVVGDPKTDQVHLGPLINDKQVARVHALVESAQKQGAKVLVGGTHQGRFYQPTVLMDVRPDMDVFKSEIFGPVAPITVFDTIDEAIELANSSEYGLAASIHTSAIATALQIAKRLKTGMVHINDQPINCEPHVPFGGMGASGTSGRFGGLSSIDEFTQSQWISMVEKPTNYPF

SEQ ID NO: 132 - protein, 487 aa, Halomonas cupida
MSTFFNAETYSNRIYLNDWRESRGGTSDVVEPATGKVLARTAIGNSEDIREAIVEAKAQQPAWARLPFDQRARILRRAAELLLEHRDTFIEWNIRECGSIVPKAEAELHSTHEQLNMAAAMTMQPDGITLPSSMPGRRNTCRRVPLGVVGVITPWNFPLLLAMRSVAPAIAVGNSVVLKPDHQSAVTGGLLIARLFEEAGLPAGVLQVIPGGAEAGEALVTHPLTAMISFTGSTAVGRKIGRTCGELLKKSALELGGNNAFIVLDDADIDAAASHGAWGAYLHQGQICMQSGRHFVHHSVAEAYISKLAERAERLTVADPFLGTADIGPLINAQQLEKLDMAVTASINDGARLVTGGHSHGQFYRPTVLSNVSIDMPAFQQELFGPVAPVTTFHDEEELIEKVSASSYGLAAAIHSSSIGRALDLAERIPAGMIHINDQTVNNEFQVPFGGFGDSGNSGRFGGPANLEEFTQSQWVSLMNTPRTYPF

SEQ ID NO: 133 - protein, 498 aa, Pseudomonas fluorescens
MTTANLHNQYPSIAEFIAEHRWKACFYPGAWESAEREIPVFEPATGERLASVGIASAAEVARAGLRARQAQPAWAATPFDQRAAILREAARLLQQEAESFIEWNIRECGGARFKAEWELNICVEQLQMAAAMPMQANGELFPSSMPGRTNIWRRVPMGVVAVISPWNFPLLLSLRSIAPALALGNAVLLKPSEFSSVTGGLLLARLFELAGVPQGVFQVLPGLAETGSALVSDPCVKMVAFTGSTAVGRRIAETCGGLLKRCSLELGGNNALIVCPDADLDAASSSGAWGSFLHQGQICMQAGRHIVHRSVVAAYTEKLKDRAERLACGNPFTEAVQLGPLINAQQRDRVHGLVQDAVHQGATLVTGGEYKELCYRPTVLIGVTPDMPVFKDEIFGPVAPIVVYDDIEEALALVNASPYGLAVAIHTGNATRGYEWAGRIHSGMVHVNDQTVNNEFQVPFGGMGASGYGGRYGGPANFDEFTERQWVSLTSDPIQYPF

SEQ ID NO: 134 - protein, 487 aa, Glaciimonas immobilis
MNTSTVTNIWDSKIYSGGWIAAEGGTAAIIEPATEQVLGHIGIGATQDVDRAVQIASHAQRSWARMPFDQRANIMREAARLVLERAAEFNVWNIRQCGSIPAKAEWELHATCEQILMAAALPMQPEGLLFPSSMPGRTNLSRQLPIGVIGVITPWNFPLLLAMRSVAPALALGNAVILKPDQQSAICGGALIAQAFEDAGLPVGVLHVIPGGPATGDALVKHPEVGMISFTGSTAVGRAIGQTCGYLLKKVALELGGNNAIIVLDDADMDAASSNGAWGAFLHQGQICMQTGRHLVHHSVADQYAEKLAARAEKLHVGNPHTDQVHLGPLINRKQCDRIHGIVQETLRAGAHALTGATHERLFYRPTVLTGVTPDMAAFQEELFGPVAPVTVFHDDDEAVELVNRSAYGLCAAIHSRNIPRAVALSQRLNTGMIHINDQTVNNEFHVPFGGMGSSGNGGRFGGPANVHEFTQSQWLSIMEKPVIYPF

SEQ ID NO: 135 - protein, 487 aa, Paraburkholderia unamae
MTGTGSEGQWTGKIFLGEWVKGTGATAPVMEPATDNQIGTIALASREDVDTAIERAVVAQRAWAETTFDKRAAVLHEAARLIKARAERFNYWNVRECGSIVPKAQWELDASYEQLLMAAALPMHPTGTLFPSSMPGRTNTWRRLPIGVVGVIAPWNFPLLLALRSVAPAIALGNAVVLKPDQQSAVTGGALIAELFEDAGLPRGVLQVLPGGAQTGDAVVRHPAVGMISFTGSTAVGRQIGETCGRMLKKTSLELGGNNPIIVLPDADLDKAASCAAWGAFLHQGQICMQAGRHLVHRSVAESYVAKLAARARKLAVGNPATEPVHIGPLINARQAERVERIVRDSVEMGAVIAAGGQRRGRFFEPTVLADVTPHMPAFKDEIFGPVAPVTLFDSVDEAIELVHASEYGLAAAVHSGSMSAAMSVARRLKSGMIHINDQTVNNEFQVPFGGMGASGNGGRFGGPANVEEFTQTQWISAMDAPIEYPF

SEQ ID NO: 136 - protein, 486 aa, Marinobacter salsuginis
MDMPASPVWQEQLFLGSWKSGDGDQINVVEPATGAVISKLKIATAGDVERAATIARDTQTAWAMVPFDQKAEILRKAAALLKERANEINDWNTRECGSVGPKADWELQATYEQAQMAAALPMQPNGEIFPSNMPGKRNYWKRVPIGTVGVIAPWNFPILLAMRSVFPALAMGNAVILKPDPKSSICGGALMAQILSDAGLPEGVFHVLPGGPEVGQALVEHPLVKMISFTGSTAVGRKIGETCGRTLKKAALELGGNNAQVVLEDADLDIASSCGAWGAFLHQGQICMQTGRHLVHTSVAEEYLSRLASRAENLACGNPAQEQVHQGPLINGVQAKRVEDIVNRSVEMGARIVTGGKRHGNYYEPTVITDVTSNMPVFSEEVFGPVAPVMTFDSDSEACELVNESPYGLAAAIHSGSTERALKIANRIQVGMIHINDQTVNNEFQVPFGGMGSSGNSGRFGGPANIEEFTTSQWISVMEEGIQYPF

SEQ ID NO: 137 - protein, 486 aa, Aromatoleum toluclasticum
MNDRNTTRWHQRIFVGEWTPGRGDTVPVIEPATGDQLALLSTASIEDVDAAARLAAEAQPAWAALPFDRRAAVLRKVAQLLQERAAEINHWNIRECGSIPPKAEWELNATIEQAHMAAAMPMQPIGEIFPSSMPGRRNYWQRLPIGVVGVIAPWNFPILLGLRSVLPALAMGNAVILKPDLQSAICGGLLLAEVFEDAGLPKGVFHVLPGGPVTGDALVRHPRVKMISFTGSTAVGRLIGETCGRMLKKVALELGGNNAMVILDDADLESASSCAAWGAFLHQGQICMQAGRHLVHRKVADRYAELLAVRAAKLVVGNPATGPVHLGPLINDRQAAKVAEVVERSAALGARVLAGGKRDGRFFPATVLAGVTPDMPAYTEEIFGPVAPITVFDSDDEAVALVNGSDYGLAVAIHSASISRAQRMATHLNAGMVHINDQTVNNEFQVPFGGMGASGNGSRFGGPASFEEFSQTQWVSVMDQGIQYPF

SEQ ID NO: 138 - protein, 496 aa, Ideonella livida
MHTPATAGPLAADDTRRWSGRLYGAAGWQPAQGGTAAVTEKATGRALAEVALANAEDVDLAARSAAAAQTAWAATPFDQRAAVLRRAEALLAERAERFAHWNVREAGSIPPKAAWEWQATREQLSMAAALPMLPVGQVFPSAMLGRRNEWRRVPLGVVGVIAPWNFPLLLAMRSVAPALALGNAVILKPDLQTPVVGGQLIAELFEDAGLPAGVLQVLPGGPATGDALVRHPQVAMISFTGSTAVGRSIGATCGGLLKKCVLELGGNNALIVLDDADLDAAASSGAWGAFLHQGQICMQAGRHLVHRSVADAYAQRLAERAARLVVGDPAAGPVHLGPLVNERQAQKVAQIVDAAVAAGARVLAGGPREGLFFPATVLTGVTPDMAAFTEEIFGPVAPITVFDTEDELVALVHQSPYGLAAAIHTRHTPRGVALAQRLHTGMVHLNDQTVNNEFHVPFGGMGASGNGGRFGGPANVEEFTQTQWISVMEQGIQYPF

SEQ ID NO: 139 - protein, 487 aa, Burkholderia_sp._D7
MNDSKQARKWEGRIFSNGWVPAAGGTAPVIEPSTGDTLAAIGMGLPEDIDRAAHSASAAQPSWAAMPFDQRAAILREAARLLKEHASEINDWNVRECGSTRAKAEWELHATYEQLHMAAAMPMQPEGALFPSALPGRMNFCRQIPIGVVGVIAPWNFPLLLAMRSVAPALAVGNTVILKPDLQSAVAGGLLLAQVLEDAGLPAGVLHVVPGGPATGDALVRHPKVGMISFTGSTAVGRAIGQICGQMLKKVSLELGGNNAIVVLDDADVDAASSSGAWGAFLHQGQICMQTGRHLVHRSLAEQYASKLAERARKLAVGDPYKAQVHLGPLINQKQRDRIDDIVRKTLASGATLLTGGRFEKLFYQPTVLTGVTTDMPAFTEEIFGPVAPVTVFDDDDEAVALVNASDYGLAAALHTRSLSRGFALSSRIRAGMVHLNDQTVNNEFHVPFGGMGSSGNGGRFGGPANVHEFTQTQWISALDKPIAYPF

SEQ ID NO: 140 - DNA, 1458 bp, Hydrogenophaga aromaticivorans
  source 1..1458: mol_type = genomic DNA
aatactccggtgaaaacggagcgttggtctggcaaaatcttcaccggcagttgggtagccgcgagaggaggcgtggcccccgtactcgaagccgcaactggggcagccttaggggaagttggcgtggcaagtccggaagacgtggatgccgcagcacgcagtgcccaagctgcccagaaagcgtgggccgcaaccccgtttgatcaacgtgcggcgattgtgcgtgaagctgcgcgtctgctgaaagaacgcgcagcggagttcacccagtggaacgttcgcgaatgtggtagcattgtccccaaaggcgaatgggaagtggggatcacccacgaacagatgcagcaagctgcggcactggccggtcttccgaatggcatgatgttcccgtcgtcggtaccgggtcggactaacctctggcaacgggtaccgcttggcgttgtcggcgtcattgccccatggaactttccgctgtttctggccatgcgttcagttgctcccgcattggcgctgggcaatgcggtacttctgaaaccggatttgcagagcgcggttacgggtggggccctgattgctcgcttattcgaggatgtcggcttaccacccggtgtcctgcaggtgctgccaggcggcccagcgacaggtgatgctgtggtgaggcatccttgcgtcaacatggtcagcttcaccggatcaacagcggtgggacgtcagataggcgagttctgtgggcgtgcgttgaagaaggttgcactcgaactgggcggcaataacgccatgattgtgctggacgatgcggatttggacggtgcctcctcttgtgcagcgtggggcggttttctgcatcagggccagatctgcatggccgcgggtcgccatctcgttcaccgttctgtcgccgatgcgtatgccgcgaaattagtggaacgcgcgaaaaagctgtacgttggagatccgcatgcaggtcctgcgcatcttggccctctgatcaatgatcgccagacggaacgtgtgcatcgcattgtaaccgagtcgattgctgcaggcgcaaccctgctagctggcggtacccacgagggtcgcttctatcagccgacggttctgagcaatgtggcggttgacatgccagcgtttgctgaagagatctttgggccggtagctccgattaccgtgtttgacacggatgaagaagcggtcgcactggccaacagctccgaatacggtttagcggccgcgatccacagcaaatcgacagctcgagcgttgcgaatggcctcccaactgaaatcaggcatggtccacatcaacgaccagcctgtgaactgcgaacctcaagtgccgtttgggggtatgggagcgagcgggagtggtggtcgctttggaggtccggcttccattgacgagtttacgcaagcgcagtgggttagcgtttctgaaaaagcagcccagtatccgttc

SEQ ID NO: 141 - DNA, 1458 bp, Pseudomonas aeruginosa
  source 1..1458: mol_type = genomic DNA
cgcgaaacgaaagaacagcccatttggtacggcaaagtgttctccagcaattgggtggaagctcgtggcggcgtagccaatgttgtggatccgtcaaatggagacattctggggattacgggcgttgctaatggcgaagacgttgatgctgcggtgaatgcggcgaaacgcgcacagaaagaatgggcggcgattccgttttctgaacgcgctgcgatcgtgcggaaagcggcagaaaagctgaaggaacgggaacacgagtttgccgattggaatgtgcgagaatgtggtgcgatacgcccgaaaggtctgtgggaagctgggattgcctacgaacagatgcaccaagcggccggactggcgtatctgtcgaacgggaccttgtttcctagtgcggtgcctggcaggatgaacctgtgccaacgtgtcccagtgggtgttgttggggtcatagcgccttggaacttcccgttgtttctggcgatgcgttcagtagcaccagcgctcgccttgggcaatgccgtgatcctgaagccggatctgcagacagccgttactggtggcgcactgattgccgagatcttttccgatgccggtatgccagatggcgtgctccatgtgttaccagggggtgcagatgttggtgagagcatggttgccaactctggcatcaacatgattagcttcaccggctctacgcaggtgggccgtctgattggcgagaaatgcggtcgtatgcttaagaaggtggcgttggaactgggtgggaacaatgtccacatcgtgttacctgatgcggaccttgatggcgcagtttcgtgtgcagcatggggcacctttctgcatcagggtcaggtttgcatggcagcgggccgccatctagtccatcgtgatgtggctcagcagtatgctgagaaacttgctttacgtgcaaaaaacctcgtcgtcggtgacccgaacagtgatcgcgttcatctgggtccgttgattaacgacaaacaggtagtacgtgtccacgcactcgtggagagcgctcaatcagcaggcgcaaaagtactggccggagggacctatcaggatcgctattaccaagctaccgtcattatggatgtcaaaccggaaatggaggtcttcaaatccgaaatcttcggtccggtagcgcccatcacagtgttcgacagcattgaagaggccattgaactggccaattgcagcgaatatggccttgccgcgtctatccatactagagcgttagcgacgggcttagatatcgcgaaacgcctgaacaccggaatggtgcacattaacgaccaacccatcaactgtgaaccgcatgtaccgtttggagggatgggctcatccggctcgggtggtcgctttggtggtctggccagcattgacgaattcacccaaagccagtggatcagtatggttgagaaatcggccagttacccgttt

SEQ ID NO: 142 - DNA, 1458 bp, Pseudomonas sp. MAP12
  source 1..1458: mol_type = genomic DNA
catgaaaccaaagaacagccaatatggggaggcaagatcttctcgagcacctgggtagaagcgcgtggtggtgtagctaacgtggtggatccctctaatggagacatcctgggcattactggcgttgcaaaccgcgaagatgtggatgtggctgtttccgcggccaaaattgcccaaaaagaatgggcagcgatgccgttttccgaacgcgcagcaattgtgcgtaaagctgccgacaaactgaaagagcgggaacacgagtttgccgattggaatgtccgcgaatgtggggcgattcgtcccaaaggcttatgggaagcgggtattacgtacgaacagatgcaccaagccgttggccttgcctcactgccgaatggtgccctgttccctagtgccgttagtggccgcatgaatctctgccagagagtcccgattggggttgtcggtgtgatagccccgtggaattttcccctgtttctggccatgcgaagcgtagcaccagcgttggttctgggcaatgcggtggtgctgaaagcggacttgcagacagccgtgattggaggtgccctaatcgctgagatcttttcagatgcgggtattccagaaggagttctgcatgtacttcctggcggtgcagacgttggcgaatcaatggtcgagaatcctggcatcaacatgatctcgttcacggggtctactcaggtcggtcgctccattggcgaaaagtgtgggcgcatgttaaagaaggtgagtctcgagttaggcggtaacaacgtcaacattgtcctcccggatgcggatcttgatggcgcagtgggttgtgcggcgtggggtaccttcttccatcagggtcaggtgtgcatggcagcgggtcgccatctggtccatcgtgatattgcgcaggaatatgcagccaaactggcgaaacgggcgcagtcactggttgtaggggatccgaacaccgaccaagtgcatctgggccctttgatcaacgacaaacaagttgatcgtgttcacgctctggtggaatctgccgaacgtgcaggtgctaaagtcctggcaggtggcgcgtatgaaggtcgctactatcaagccaccgtagtgatggatgtcaaaccggacatggagattttccagagcgagatctttggcccggttgccccaatcacgattttcgacagcattgatgaagctatcgaattggcgaattcgtccgaatatggcttagcggctagcatccacacgaaatcgctcaccaccgggatgaagatcgcgaatcgtctgaaaacgggtatggtgcacattaacgatcaaccgatcaactgcgaaccgcatgtaccgtttggcggcatgggggcatctggcagtggaggacgttttgggggcactgctagcatcgaggagtttacccagagccagtggattagcgtggtggacaaaacagcggtttacccgttt

SEQ ID NO: 143 - DNA, 1464 bp, Alteromonas
  source 1..1464: mol_type = genomic DNA
caacaggaacgtaagaaggaagtgccgatttggtcggggaaagtcttctcctcagggtgggtggaagcgcgtggtggcgcgtctgatgtgaccgatccgagcaacggtgatctcctgggcgtggtgggcattgcgaatggcgaagacgttgccgcggccgcacagagtgctcgcagagcgcagaaagaatgggctgcgattccgtttagcgaacgcgccgaaattgtcaggaaagcggccgaaaaactgaaagaacgcgaaaatgagttcgcggattggaacgttcgggaatgtggtgcgatccgccagaaaggcctgtgggaagctggtatcacctatcagcagatgcaccaagcggcaagtctcgcttttctcccagatgggacgagtttaccctccactgtggctggtcgcctgaacttgtgccatcgtgtgccggttggggtagtaggcgtcattgcgccgtggaattttccgctgttccttgcgatgcgatccgtagctccagcactagtactgggcaatgcggtcattctgaaaccggatcctcagactgccgttacgggtggtgcattgattgcggagatcttctctgaagccggcattcctgatggtgtgatccatgtgctaccaggaggagcggaagctggcgaatcgatggtaaccaatccggggattgacatgatctcgttcacagggagcacagaagtcggacgcttaatcggggagaagtgtggacgtatgctgaagaaagtggcactggagttaggcggcaataacgtccacatcatcctgccggatgcagacctggatggcgcagcgtcttgtgcagcctggggtacctttctccatcaaggccaggtttgcatggcagcgggtcgtcacttagtccaccgtgacatagcccaggaatatgcggagaaactggcactgcgtgcccgtaacctggttgtcggtgatcccaaaacggaccaggttcatcttggcccgttagttaacgacaaacaggtggcgcatgtgcatgctctggtggagagcgcccaaaaagccggcgcaaaaattctggctggtggaacttaccaagatcgctattaccaagcgaccgttcttatggatgtcacccctaagatggacatcttcgagttggaaacgtttggtccagttgccccgattaccatcgttgactctgtggaagaggccattggcctggccaattcgagcgaatacggtttggcagcaagcatccacacgaaagatcttgctgcgggtttggagatagcccgcaacctgaaaacaggcatggtgcacattaacgatcagccgattaactgcgaaccacatgtaccctttggtggcatgggtgcctcagggtcatccggccggtttggaggcctggcgagtatcgacgcgtttacccaaagccagtggattagcatggtgggcaaacctgccacctatccgttt

SEQ ID NO: 144 - DNA, 1458 bp, Tepidiphilus succinatimandens
  source 1..1458: mol_type = genomic DNA
aactggaatggcaaattgccgatatggcatggcaaagtgttctccaatgggtgggtcgttcctagaggtggagttgcggacgtagtggatcccagtagtggcgatgtactgggtgttaccggcatagcgaacagcgaagatatcgctaccgccgcatctgcggcgaaagaagcccagaaaaagtgggcggccatgccgttcaatgatcgagcggccattttgcggaaagccgccgaaaaactgcgtgaacgcgaagcggaattcgcagattggaatgttcgcgagtgcggtgctgtacgcatgaaaggcgtgtgggaagcggggattacctacgaacagatgcaccaagctgcgtcgctagcctttctccctaatggaacgttgtttccatcacaggtgccaggccgtatgaactttgtgcatcgcgttccggtgggtgttgtgggcgtgattgccccgtggaattttcccctgttcctggcgatgcgcagcgttgcaccagcattggttcttggaaatgcggtcattctgaagcctgacgtccagacagctgtgaccggtggtgcgctgatcgcagagatctttgcagaagcaggcattccggaaggtgtcttacatgttctcccgggtggtgccgatgcgggcgacgcgatggtcaccaatccggagattgacatgatttccttcactggcagcactgctgtgggtcgtcagattggcgagaaatgcggccgtatgctgaagaaggtgacgctggaactgggtgggaacaacgtgcacattgtcctgccggacgccgatctgaccggtgcagcttcgtgtgcagcatgggggacgtttctgcaccaagggcaggtttgtatggctgctggccgtcatctggtgcaccgcgatgttgcccagcaatatgcgcaggagttagccgcacgtgccaaaaacctcgtagttggcgatcccaaaaccgatcaggtccatcttggcccgctgatcaacgacaaacaagtcgctcgcgtgcatgcgcttgtcgaaagtgcgcagaaacaaggtgcgaaagtgctcgtaggagggacgcatcaaggccgcttttaccagccaacagttctgatggatgtacgtccggacatggacgtcttcaagtctgagatcttcggtcctgtggcaccgatcaccgtgtttgatacgattgatgaggcgatcgaactggccaatagcagcgaatatggcttagcggctagcatccatacctccgcaattgccactgcgcttcaaattgccaaacggctgaaaacaggcatggtgcacatcaacgatcagccgattaactgcgaaccacacgtaccgtttggcgggatgggtgcgtcaggtacttcgggtcgttttggcggattatcgtcaatcgacgaattcacgcagagtcagtggatctctatggtcgaaaaacccaccaactatccgttt

SEQ ID NO: 145 - DNA, 1458 bp, Halomonas cupida
  source 1..1458: mol_type = genomic DNA
tcgacctttttcaacgcggaaacgtacagcaatcgcatctacctgaatgattggcgggaaagtcgcggtggtacaagcgatgtggtggaaccggcgacaggcaaagtcctggcgagaaccgctattgggaactccgaggatatccgggaagcgattgtggaagccaaagctcagcaaccggcatgggcgaggttacccttcgaccaacgagcccgcattctgcgccgtgccgctgaattgttgctggaacaccgtgacacctttatcgaatggaacatccgcgaatgcggctctatagtcccgaaagcggaagccgaacttcactcgacgcacgaacagctgaacatggcggcggctatgactatgcagccagatggcattaccctgccgtcaagcatgcctggtcgccgtaatacctgtcgtcgagtgccgttaggcgtagtcggagtcatcacaccgtggaactttccgttgctgctggccatgcggtccgttgcgccagcaattgccgttggcaatagcgtggttctgaaaccggatcatcagagcgcagtgaccggtggtttgctgattgcccgcttattcgaggaagcgggcttaccggccggggtactgcaagtcattcccggaggcgcggaagcaggtgaagcccttgtgacgcatccactcaccgccatgatctcctttactgggagtactgcggtaggtcgcaaaatcgggcgtacatgtggggagctgctgaagaaaagtgcccttgaactgggtggcaataacgcgttcattgtgctggatgatgccgacattgatgcggcagcatcccatggtgcttggggagcctatctgcatcaaggccagatatgcatgcaatcaggccgtcactttgtccaccattctgtcgctgaggcgtatatcagcaagttagctgaacgcgcagaacgccttaccgtggcggatcccttcttaggcactgcagacatcggcccgctgattaacgcgcaacagctcgagaaactggatatggccgttacggcgtcaattaacgacggagcccgtctagttacgggtggtcattcccatggacagttctatcgtccgacggtgctgagcaatgtgtcgattgatatgccagcgtttcagcaggagctctttggcccagtagcaccggttaccacctttcatgacgaagaagagctgatcgagaaagtgtctgcttcatcgtatggcctagcagcggcaatccattcgagctctattggtcgtgcgttggatctcgccgagcgtattccggctggcatgattcacatcaacgaccagaccgtaaataacgagttccaggttccttttgggggttttggtgatagtggcaatagtggccgctttggtggccctgcaaatctggaagaattcacgcaaagccagtgggtttctttgatgaacactccgcgtacctaccctttc

SEQ ID NO: 146 - DNA, 1491 bp, Pseudomonas fluorescens
  source 1..1491: mol_type = genomic DNA
accaccgctaacctgcacaaccagtacccgtcgattgccgagttcatcgcggaacaccgttggaaagcgtgcttttatccgggtgcctgggaaagtgccgaacgtgagatccccgtttttgagccagcaacgggtgagcgtctagcgagcgtcggaattgctagtgcagccgaagtagctagggcgggattgcgcgcacgccaagcgcaaccagcatgggcagccaccccatttgaccagcgtgcggcgatcttacgcgaagcagcgcgtcttctgcaacaggaagccgaaagcttcatcgagtggaatatccgggaatgcgggggtgcccgtttcaaagccgaatgggaactcaacatatgcgtagagcagctgcagatggctgctgcaatgcccatgcaagccaatggggaacttttcccgtccagcatgccaggacgcaccaacatttggcgaagagtgccgatgggagtagtggcggtgattagtccgtggaactttccgctcctgttgtcgttgcgctccattgcccctgctctcgcacttggcaatgccgtcttgctgaaaccgtcagagttcagctctgtgactggcggtctgctgttagcgcgtctgtttgagctggctggcgttccgcaaggtgtctttcaggtcttacctggtttagccgaaacgggttctgccctggtatcggatccctgcgtcaaaatggtggcatttacgggctcaacagcggttgggcgccgcattgcagaaacttgtggcggcttactgaaacgctgttccctggaactgggtggtaacaacgcgctgattgtgtgtcccgatgcggaccttgatgctgcctccagttctggcgcatggggcagcttcctgcatcagggccagatttgcatgcaggcgggccgccacattgtgcatcgaagcgttgttgctgcctacacggaaaagctgaaagatcgcgcggaacgtctggcgtgtgggaatccttttaccgaagcggtacaactgggtccgctgattaatgcacagcaacgcgatcgggtccatggtttggtccaggatgcggtgcatcaaggcgcgacgttggtgacagggggtgagtacaaagaactctgctatcgccctaccgtactgataggcgtgactccggatatgccggtcttcaaggacgaaatctttggcccagtggcgcctatcgttgtgtatgatgacatcgaagaagctctggcgctagtgaatgcgagcccgtatggcttagcagtggccattcacaccggcaatgccacacgtggttacgaatgggcaggccgtatccattcgggcatggttcatgtgaacgaccagacggttaacaacgagttccaggttccgttcgggggtatgggcgcctcaggttacggaggccggtatgggggtccggcgaattttgacgagtttaccgaacgtcagtgggtttctctgaccagcgatccgattcagtatccgttt

SEQ ID NO: 147 - DNA, 1458 bp, Glaciimonas immobilis
  source 1..1458: mol_type = genomic DNA
aacaccagtaccgtaacgaacatttgggacagcaagatctactcaggcggttggattgccgccgaaggcggaactgccgccatcattgaaccggcaacagaacaggtgctgggacacattggcatcggcgcaactcaggacgttgatcgcgcggtgcagattgccagtcatgcccagaggtcttgggcgcgtatgccgtttgaccaacgcgcgaacattatgcgggaagctgcgcgtttagtgctggagagagctgcggagttcaatgtgtggaacattcggcaatgcggatctatccccgctaaagcggagtgggaactgcatgctacctgtgagcagattctcatggcagctgcgttaccgatgcaaccggaaggcttgctgtttccgagcagcatgccagggcgcacgaacctgtcgcgtcaactgccgattggcgtgataggcgtgatcaccccttggaactttccgctgctgctggccatgcgctcggtagctcctgccttagcactgggtaatgcggtgatccttaaaccggatcaacagagtgccatttgtggtggtgcactcattgctcaagctttcgaagatgcaggccttcctgtgggcgttctgcatgtgattccaggcgggccggccactggcgatgctctagtgaaacatccggaagtcggcatgatttcgtttaccggttcaaccgcggtcggtcgagcgattgggcaaacgtgtgggtacctcttgaagaaagtggccttagaactggggggtaataacgcgatcatcgtcttggatgatgcggatatggatgccgcgtcttccaatggggcgtggggtgcattcctgcaccagggccagatttgcatgcagacaggtcgtcatctagtccatcactccgttgccgaccagtatgcagagaaattggcggctcgtgcggaaaaactgcacgtaggcaatccccataccgatcaagtgcatctgggtccgctgattaaccgcaaacagtgcgaccgcatccacggtatcgtccaggaaacccttcgtgcgggcgcacatgcactgaccggtgccacccatgaacgcctgttctatcgtccaacggttttaacgggcgtaacaccggatatggcagcgtttcaggaggaactgtttggcccagttgcgccagttacggtattccacgatgatgacgaagccgttgaactggttaatcgtagtgcctatggcctttgcgcagcaatccattcgcgcaacataccccgtgcggtggcgttgtcccagcgcctcaatacgggtatgatccacattaatgaccagaccgtcaacaacgagttccacgttccctttggaggcatggggagctcaggcaacggtggacgctttggtggtccggcgaatgtccacgaattcactcagagccaatggctgagcatcatggaaaaaccggtcatctaccctttt

SEQ ID NO: 148 - DNA, 1458 bp, Paraburkholderia unamae
  source 1..1458: mol_type = genomic DNA
acggggactggcagcgaaggccaatggaccggcaagatcttcctgggcgaatgggtcaaaggaacgggtgcaacagccccggtgatggagcctgctacagacaatcagattggtaccattgccctggccagtcgagaagacgtggacacagccatagagcgcgcagtggttgcgcagcgtgcctgggctgagacgacgtttgacaaacgagcggcagtgttgcacgaagcggcacgcctgattaaggcccgtgcagaacgcttcaactactggaacgtgcgcgaatgcggcagcatcgtgccgaaagcgcagtgggaactggatgccagctatgaacagctactgatggctgctgcgttaccgatgcacccgactgggacgttattcccctcaagcatgccaggtcgcaccaatacctggcgccgcttaccgattggtgtcgtgggcgtaattgcgccgtggaactttccgctgctcttggcactgcggtcagttgcaccggccattgcactgggcaatgccgtcgtcctgaaacccgatcagcagagtgcggtgactggtggcgcactgatcgcggaactgttcgaagatgccggtcttcctcgtggcgtgctgcaggtgttacccggtggggcccagaccggtgatgcggtagtccgtcatccggcagttgggatgatcagcttcactggatctaccgccgttggtcgccaaatcggcgaaacctgtgggcgcatgctgaagaaaaccagtttggaactgggtggcaataacccgattatcgtgcttcctgatgctgatctcgataaagcggcatcatgtgccgcatggggcgcgtttttgcaccaagggcaaatctgcatgcaagccggcaggcatctggtgcatcgctctgttgcggaaagctacgtggctaaacttgcggctcgtgcccggaaactcgcggttggaaacccagcgaccgaacccgttcacattggtcctctcattaatgcgagacaggcagaacgcgtcgaacggatagttcgtgattccgtcgaaatgggcgctgtaattgccgcggggggacaacgtcgtggtcgctttttcgaaccgacagttctggcggatgtcaccccgcatatgccagcgtttaaagacgagatttttggaccagtagctccggtgacgctgttcgattccgtagacgaagccatcgagttagtgcatgcctcggaatatggccttgcagcggcggtgcattcgggctctatgagtgcggcgatgtcggttgcacgtcgtctgaaatccggtatgatccacattaacgaccaaacggttaacaacgagttccaggtaccgtttggcggcatgggtgcttcgggtaatggcggccgttttggtggtccagcgaatgtcgaggagtttacccagacccagtggatcagcgctatggatgcccctattgagtatccgttt

SEQ ID NO: 149 - DNA, 1455 bp, Marinobacter salsuginis
  source 1..1455: mol_type = genomic DNA
gatatgccagctagcccagtatggcaagagcagctctttttaggctcctggaaaagtggggatggtgatcagatcaacgtagtggaacctgcaacaggtgcggtcatctcgaagctgaagatagcgaccgcaggggatgtggaacgcgcagcaacgattgcacgcgacacccagactgcgtgggctatggtgccgttcgatcagaaagcggaaatcctccgcaaagcggcggcgctgctgaaagagagagccaacgagatcaatgactggaatacgcgggaatgcggttcggtaggaccgaaagcggactgggaactgcaagcgacctatgaacaggcccagatggctgcagcattgccgatgcagccgaatggcgaaatcttcccatcaaacatgcccggcaaacgcaactattggaaacgtgtccccattggtaccgtgggtgttattgcgccatggaatttcccgattctgctcgcgatgcgtagcgtgttcccagctttggccatgggaaatgccgtgattctgaaaccggatcccaagagctccatttgtggcggtgctcttatggcccagattctgagcgatgcaggcttaccggaaggcgtgttccacgttctgcctggtggcccggaagttggccaagcgttagtggaacatccgctggtgaaaatgatttcctttacgggctctactgcggtcggacgcaagatcggcgaaacatgcggtcgaaccctgaaaaaagcggctctggaattgggtgggaacaatgcccaagtcgttctggaagatgccgaccttgacatcgctagtagctgtggtgcctggggcgcctttctgcatcaagggcagatttgcatgcagactggtcgtcacctagtgcatacgtcggttgccgaggaatacttgagccgtcttgccagtcgcgcagaaaacctggcctgtggtaatcctgcacaggaacaagtgcatcaggggccgctgattaatggcgttcaggccaaacgggtagaggatattgtcaatcgctcagtagagatgggagcacgcatagtcactggtggcaaacgtcatggcaactactacgaaccgaccgttatcaccgatgtgacctccaacatgccggtttttagcgaggaagtgtttggcccggttgccccggtgatgaccttcgacagtgattcggaggcttgcgaactggtgaacgaatctccctatggcttagctgcggcgattcacagtggttctacggagcgtgcgctcaaaatcgcgaaccgtatccaagtcggcatgattcacattaacgaccagacggtaaacaacgagtttcaggttcctttcggaggtatggggtcgtcagggaattctggccgttttggtggccctgcgaatatcgaagagtttaccacatcacaatggatcagcgtcatggaagaaggcattcagtatccgttt

SEQ ID NO: 150 - DNA, 1455 bp, Aromatoleum toluclasticum
  source 1..1455: mol_type = genomic DNA
aacgatcgcaatactacgcgctggcatcaacgcatctttgtaggcgaatggacaccgggtcgtggtgacacggttccggtgattgagccagctacgggcgatcaactggcgctgctcagtaccgcgtcgattgaggatgttgatgcagcagcgcgtctagctgccgaagcacagccagcttgggcggcactgccctttgatcgtcgcgcagcagtcctgcgcaaagttgcccaactgctgcaagaacgcgcagcggaaatcaaccactggaacatccgtgaatgcggcagtattccgccgaaagcggaatgggagctgaatgcaaccatcgaacaggcccatatggccgcagccatgcctatgcagccgattggtgagatctttccctcgagcatgcctggtaggcgcaactactggcagcgtctgcctattggtgtggttggcgtcattgccccctggaactttccgatcttgctgggccttcgcagcgtattgccggcgttagctatggggaatgcagtcattctcaaaccggacttacagagcgcgatttgcggaggcctgttgctggccgaagtgttcgaagatgctggcctgcctaaaggggtcttccacgtactgccgggtggcccagttacgggtgatgccctggtgcgtcatccccgtgtcaagatgatcagctttaccggtagtaccgcggtcggccgcttgattggcgaaacctgtggtcgtatgctgaagaaggtagcgctcgaactgggcgggaacaatgccatggtcatacttgacgatgctgatcttgaaagcgcctcttcctgtgctgcatggggcgcgtttctgcatcaagggcagatttgcatgcaggctggtcgtcatttagtgcatcgcaaagtagccgaccgctatgccgagttgctggcagtgcgtgcggctaaactggtggttggtaatccggcgacaggtccggtgcacttagggccgttaatcaacgatcggcaagccgcgaaagttgcagaagtcgtagaacggtcagcggcgttaggtgcgcgagtgctagcgggtggaaaacgtgatggccggttctttccggccactgtgcttgcaggagttaccccagatatgccggcttatacggaagaaatcttcggcccagtggcgccgattaccgtgttcgactctgacgacgaagcggttgcgctggtcaatggatccgattatggcctggctgttgccatccattccgccagtatatctcgagcgcagagaatggcgacacacctcaacgccggaatggtgcacattaacgaccaaaccgtgaataacgagtttcaggtgccgtttgggggcatgggtgcgtcaggcaatggctcacgctttggcggtcctgcctcgttcgaggagttctcgcagactcagtgggttagcgtgatggatcaggggattcagtacccattc

SEQ ID NO: 151 - DNA, 1485 bp, Ideonella livida
  source 1..1485: mol_type = genomic DNA
catactccagccactgcgggcccactggctgcggacgatacgaggcgctggagtggtcgcttgtacggtgcagcagggtggcagccggcgcaaggtggtacggctgctgtgaccgagaaagccacaggccgagccttggcggaagtagctctggctaatgcggaagacgtcgatttagcagcacgtagtgctgcagctgcccagacggcatgggcagcgactccgtttgatcagcgtgcagcggtccttcgccgtgcggaagccctgttagccgaacgcgcggaacgtttcgctcactggaatgtgcgtgaagccggctcgattccccctaaagcggcttgggaatggcaagcgacacgggagcaactcagcatggcggctgcactaccgatgctgcctgtaggccaggtttttccgtccgcgatgctggggcgccggaacgagtggcgtcgcgttccattgggcgttgtcggggtcatcgcaccctggaactttccgctgctgctcgccatgcgttcggtggcaccggcccttgcgctgggaaatgccgttatcctaaaaccggatcttcaaaccccagtggttggcggtcagctgattgccgagctgttcgaagatgccggtctgccggctggtgtgctgcaggtattgccggggggcccagcgaccggtgatgccctcgtccgtcatccccaggttgcgatgattagcttcaccggctctaccgccgtcggtagatcaattggggctacctgtggcggcctgctgaagaaatgcgtgcttgaactgggcggcaacaatgcgctgattgtcctcgatgatgccgacctggatgcagcggcctctagcggagcgtggggtgcgtttctgcaccagggccagatctgcatgcaagcaggtcgccatctggtccatcgatcggtagccgacgcgtatgcgcaacgtcttgcggaacgcgcagcacgtctggtagttggcgatcctgccgccggtccggtgcatctcggaccgttagtcaacgaacgtcaggcgcagaaagttgcgcagatagtggatgccgcggtagctgcgggtgcacgtgtgttagcgggaggtccacgcgaaggcctgttcttcccggccacagtgttaaccggagttaccccggacatggcggcgtttaccgaggagatctttggaccggttgctcccatcaccgtgtttgatacggaagacgaattggtggccttagtgcatcagtccccgtatggtctggcggcagcaattcacacgcggcacacacctcgcggtgtggcattggcgcaacgcctgcatacgggcatggttcacctgaacgaccaaactgtgaacaacgaattccacgtaccgtttgggggcatgggcgcctcagggaatggcggtcgctttggcggccctgccaatgtggaggaattcacccagacgcagtggatcagcgtcatggaacaagggattcagtacccgttt

SEQ ID NO: 152 - DNA, 1458 bp, Burkholderia_sp._D7
  source 1..1458: mol_type = genomic DNA
aacgacagcaaacaggcacgtaagtgggaaggccgcattttcagcaacggttgggtgccagcagcaggtggcactgcccctgtgatcgaaccttcgaccggtgatacgttagcggcgatcggcatgggcttaccggaggatattgatcgtgcagcccattcggctagcgccgcccaaccgagttgggctgcgatgccgtttgaccagcgtgccgccattctgcgtgaagccgcgcgcttactgaaagaacatgcgtccgaaatcaacgattggaatgtccgcgaatgtgggtctacgcgcgctaaagcggaatgggaacttcacgcaacgtatgagcagctccacatggcggccgcaatgcccatgcaacccgaaggcgctctttttccttcggcactgccaggacgcatgaacttttgccgccaaattccgattggcgttgttggcgtcattgccccgtggaacttcccgctcctgttggccatgcgctcggttgcgcctgccctggcggtgggtaacaccgtcatcctgaaaccggatctccagtctgcggtggcgggaggcctactgcttgctcaggttctggaagatgccggtcttccagcaggtgttctccatgtggttcccgggggaccagctacaggggatgcgctagtcagacatccgaaagtgggcatgatcagctttacgggcagcactgcggtaggccgggcaattgggcagatatgtgggcagatgctgaagaaggtaagcctggaactgggtggcaacaatgcgattgtcgtgctggatgacgcggatgttgatgccgcgagtagttcaggcgcttggggagcgttcctccaccagggtcagatctgcatgcaaaccgggcgacatctggtgcatcgtagcttggcagaacagtacgcttcaaaactggccgaacgtgcgcgcaaattggcagttggcgatccgtacaaagcccaagtccacttaggtccgctgatcaaccagaaacaacgcgacaggatcgatgacatagtacgcaaaactctggcatcaggtgcgactctgctgacaggtggtcgtttcgagaagttgttctaccagcctaccgtattaacgggggtaaccacagacatgccggcgtttaccgaggagattttcggtccggttgctccggtaaccgtgtttgacgatgacgatgaagcagtggcgttagtcaatgcctccgattatggtctggcagctgcgttgcatacccggtcactgagtcgaggctttgcgctgtcctcccgtattcgtgctggcatggtgcacctgaatgatcaaaccgtgaacaatgagttccacgtgccctttggaggtatgggctctagcggcaatggcggtcgttttggtggcccagcgaatgtccatgagttcacccagacgcagtggatttctgccttggacaaaccgatcgcctatccgttt

SEQ ID NO: 153 - DNA, 30 bp, synthetic construct
  source 1..30: mol_type = other DNA
caccatcacggatccaatactccggtgaaa

SEQ ID NO: 154 - DNA, 38 bp, synthetic construct
  source 1..38: mol_type = other DNA
cagctaattaagcttttagaacggatactgggctgctt

SEQ ID NO: 155 - DNA, 30 bp, synthetic construct
  source 1..30: mol_type = other DNA
caccatcacggatcccgcgaaacgaaagaa

SEQ ID NO: 156 - DNA, 39 bp, synthetic construct
  source 1..39: mol_type = other DNA
cagctaattaagcttttaaaacgggtaactggccgattt

SEQ ID NO: 157 - DNA, 30 bp, synthetic construct
  source 1..30: mol_type = other DNA
caccatcacggatcccatgaaaccaaagaa

SEQ ID NO: 158 - DNA, 40 bp, synthetic construct
  source 1..40: mol_type = other DNA
cagctaattaagcttttaaaacgggtaaaccgctgttttg

SEQ ID NO: 159 - DNA, 30 bp, synthetic construct
  source 1..30: mol_type = other DNA
caccatcacggatcccaacaggaacgtaag

SEQ ID NO: 160 - DNA, 39 bp, synthetic construct
  source 1..39: mol_type = other DNA
cagctaattaagcttttaaaacggataggtggcaggttt

SEQ ID NO: 161 - DNA, 30 bp, synthetic construct
  source 1..30: mol_type = other DNA
caccatcacggatccaactggaatggcaaa

SEQ ID NO: 162 - DNA, 40 bp, synthetic construct
  source 1..40: mol_type = other DNA
cagctaattaagcttttaaaacggatagttggtgggtttt

SEQ ID NO: 163 - DNA, 30 bp, synthetic construct
  source 1..30: mol_type = other DNA
caccatcacggatcctcgacctttttcaac

SEQ ID NO: 164 - DNA, 38 bp, synthetic construct
  source 1..38: mol_type = other DNA
cagctaattaagcttttagaaagggtaggtacgcggag

SEQ ID NO: 165 - DNA, 30 bp, synthetic construct
  source 1..30: mol_type = other DNA
caccatcacggatccaccaccgctaacctg

SEQ ID NO: 166 - DNA, 39 bp, synthetic construct
  source 1..39: mol_type = other DNA
cagctaattaagcttttaaaacggatactgaatcggatc

SEQ ID NO: 167 - DNA, 30 bp, synthetic construct
  source 1..30: mol_type = other DNA
caccatcacggatccaacaccagtaccgta

SEQ ID NO: 168 - DNA, 40 bp, synthetic construct
  source 1..40: mol_type = other DNA
cagctaattaagcttttaaaaagggtagatgaccggtttt

SEQ ID NO: 169 - DNA, 30 bp, synthetic construct
  source 1..30: mol_type = other DNA
caccatcacggatccacggggactggcagc

SEQ ID NO: 170 - DNA, 39 bp, synthetic construct
  source 1..39: mol_type = other DNA
cagctaattaagcttttaaaacggatactcaataggggc

SEQ ID NO: 171 - DNA, 30 bp, synthetic construct
  source 1..30: mol_type = other DNA
caccatcacggatccgatatgccagctagc

SEQ ID NO: 172 - DNA, 39 bp, synthetic construct
  source 1..39: mol_type = other DNA
cagctaattaagcttttaaaacggatactgaatgccttc

SEQ ID NO: 173 - DNA, 30 bp, synthetic construct
  source 1..30: mol_type = other DNA
caccatcacggatccaacgatcgcaatact

SEQ ID NO: 174 - DNA, 39 bp, synthetic construct
  source 1..39: mol_type = other DNA
cagctaattaagcttttagaatgggtactgaatcccctg

SEQ ID NO: 175 - DNA, 30 bp, synthetic construct
  source 1..30: mol_type = other DNA
caccatcacggatcccatactccagccact

SEQ ID NO: 176 - DNA, 39 bp, synthetic construct
  source 1..39: mol_type = other DNA
cagctaattaagcttttaaaacgggtactgaatcccttg

SEQ ID NO: 177 - DNA, 30 bp, synthetic construct
  source 1..30: mol_type = other DNA
caccatcacggatccaacgacagcaaacag

SEQ ID NO: 178 - DNA, 39 bp, synthetic construct
  source 1..39: mol_type = other DNA
cagctaattaagcttttaaaacggataggcgatcggttt

SEQ ID NO: 179 - DNA, 39 bp, synthetic construct
  source 1..39: mol_type = other DNA
aagaggagaaattaactatgcgtgagaccaaggagcaac

SEQ ID NO: 180 - DNA, 41 bp, synthetic construct
  source 1..41: mol_type = other DNA
aagctcagctaattaagcttttacgcttcttcgacacttac

SEQ ID NO: 181 - DNA, 25 bp, synthetic construct
  source 1..25: mol_type = other DNA
catagttaatttctcctctttaatg

SEQ ID NO: 182 - DNA, 22 bp, synthetic construct
  source 1..22: mol_type = other DNA
aagcttaattagctgagcttgg

SEQ ID NO: 183 - DNA, 40 bp, synthetic construct
  source 1..40: mol_type = other DNA
aagaggagaaattaactatgaacaggttaccttcgagcgc

SEQ ID NO: 184 - DNA, 22 bp, synthetic construct
  source 1..22: mol_type = other DNA
ggtatatctccttcttattacg

SEQ ID NO: 185 - DNA, 41 bp, synthetic construct
  source 1..41: mol_type = other DNA
taagaaggagatataccatgatcataggggttcctaaagag

SEQ ID NO: 186 - DNA, 40 bp, synthetic construct
  source 1..40: mol_type = other DNA
catggtatatctccttcttattaagcacccgccacagatg

SEQ ID NO: 187 - DNA, 44 bp, synthetic construct
  source 1..44: mol_type = other DNA
taagaaggagatataccatgacgaatactctggatgttttaaaa

SEQ ID NO: 188 - DNA, 20 bp, synthetic construct
  source 1..20: mol_type = other DNA
ttaagcacccgccacagatg

SEQ ID NO: 189 - DNA, 22 bp, synthetic construct
  source 1..22: mol_type = other DNA
taagaaggagatataccatgac

SEQ ID NO: 190 - DNA, 36 bp, synthetic construct
  source 1..36: mol_type = other DNA
gtggcgggtgcttaataagaaggagatataccatgc

SEQ ID NO: 191 - DNA, 20 bp, synthetic construct
  source 1..20: mol_type = other DNA
cacttattcaggcgtagcac

SEQ ID NO: 192 - DNA, 22 bp, synthetic construct
  source 1..22: mol_type = other DNA
atcggcattttcttttgcgttt

SEQ ID NO: 193 - DNA, 20 bp, synthetic construct
  source 1..20: mol_type = other DNA
ccaattgacttcggcaagtg

SEQ ID NO: 194 - DNA, 43 bp, synthetic construct
  source 1..43: mol_type = other DNA
gtgctacgcctgaataagtggggttattccttatctatctaat

SEQ ID NO: 195 - DNA, 43 bp, synthetic construct
  source 1..43: mol_type = other DNA
acgcaaaagaaaatgccgatgaggtaaaagaataatggctatc

SEQ ID NO: 196 - DNA, 20 bp, synthetic construct
  source 1..20: mol_type = other DNA
gtcgcgtgaacataagcgtc

SEQ ID NO: 197 - DNA, 46 bp, synthetic construct
  source 1..46: mol_type = other DNA
gatagccattattcttttacctcgggttattccttatctatctaat

SEQ ID NO: 198 - DNA, 46 bp, synthetic construct
  source 1..46: mol_type = other DNA
attagatagataaggaataacccgaggtaaaagaataatggctatc

SEQ ID NO: 199 - DNA, 20 bp, synthetic construct
  source 1..20: mol_type = other DNA
ttaaaacgggtagttcgccg

SEQ ID NO: 200 - DNA, 38 bp, synthetic construct
  source 1..38: mol_type = other DNA
aactacccgttttaataagaaggagatataccatgatc

SEQ ID NO: 201 - protein, 546 aa, Arthrobacter chlorophenolicus
MHIDNIENLSDRGFDYVVIGGGSAGAAVAARLSEDPDVSVALVEAGPDDRNIPEILQLDRWMELLESGYDWDYPIEPQENGNSFMRHARAKVMGGCSSHNSCIAFWAPREDLDEWESKYGATGWNAANAWPLYKRLETNQDAGPDAPHHGDSGPVHLMNVPPADPSGVALLDACEEAGIPRARFNTGTTVVNGANFFQINRRGDGTRSSSSVSYIHPIIERDNFTLLTGLRARQLVFDADKRCTGVEVVDGAFGRTHRLTARHEVILSTGAIDSPKLLMLSGIGPAEHLAQHGIEVLVDSPGVGENLQDHPEGVVQFEAKQPMVQTSTQWWEIGIFTPTEDGLDRPDLMMHYGSVPFDMNTLRHGYPTTENGFSLTPNVTHARSRGTVRLRSRDFRDKPMVDPRYFTDPEGHDMRVMVAGIRKAREIAAQPAMSAWTGRELSPGVGAQTDEELQDYIRKTHNTVYHPVGTVRMGADDDGMSPLDARLRVKGVTGLRVADASVMPEHVTVNPNITVMMIGERCADLIKADYAGADALEEKELTTSFA

SEQ ID NO: 202 - DNA, 1638 bp, synthetic construct
  source 1..1638: mol_type = other DNA
atgcacattgacaacattgaaaacctgtcggatcgtggcttcgactacgtagttatcggtggtggcagcgctggcgccgcagttgccgcacgtctgagcgaagatccggacgtcagcgtagccctggtggaagctggtccggatgatcgtaatatccccgaaatcctgcagttagatcgctggatggaactgctggaaagtggttatgactgggattatccgattgaaccgcaagaaaacgggaactcgtttatgcgtcatgctcgcgcaaaggtgatgggtggctgttcatcgcataactcctgcatcgcgttttgggcacctcgcgaagatctcgacgaatgggagagcaaatatggggcaactggctggaatgcggcgaatgcatggccgctctacaaacgcttggaaaccaatcaggatgctggtccggatgcgccgcatcacggtgacagtgggccagtccatctgatgaacgtccctcctgcggacccatcaggagttgcgctcctggacgcgtgcgaagaagctggcattccgcgtgcacgttttaacaccggcacgaccgttgtgaatggtgccaacttcttccagatcaatcgccgtggcgatggtacgcgttcgtcgtcatccgtgtcttacattcacccgatcattgaacgcgacaactttacccttcttaccggattacgggcacggcaactggtgtttgatgcggataaacgctgcactggtgtggaagtggtggatggcgcctttggtcgcactcatcgcttaacggcgcgtcatgaggtgatcctgagtacgggtgccattgactctccgaaattgctgatgctgagtggcattggccccgccgagcatctggcccaacatgggattgaagtgttagtggattcccctggcgttggggagaatctgcaagaccacccagaaggagtcgttcagtttgaggccaaacagccgatggtacagacaagcacgcagtggtgggagattggcatcttcacgccgacagaagatggcctggatcgcccagacctgatgatgcactatggctcagtcccattcgacatgaacactttgcggcatggctatccaaccaccgaaaacggctttagccttacgccgaatgtcactcatgcccgcagtcgtggaacggttcgcctgcgttctcgtgactttcgcgataaacctatggttgacccgcgctatttcaccgatccggagggtcacgatatgcgcgtgatggttgcgggtatccggaaagcgcgtgaaattgcggcacaaccggccatgagcgcgtggactgggcgtgagctttctccaggtgttggcgctcagaccgatgaggagttgcaggattacatccgcaaaacgcataacaccgtgtatcaccccgtcggtaccgtccgcatgggtgcggatgatgatggcatgagcccgttagacgctcgcctccgcgtgaaaggggtgacaggattgcgcgtagctgatgcgtccgtcatgccggaacacgtaaccgtaaatcccaatattaccgttatgatgattggggaacgttgtgccgatctgattaaggcggattacgcaggcgcggatgcgctggaggaaaaggaactgacaacctccttcgcc

SEQ ID NO: 203 - DNA, 37 bp, synthetic construct
  source 1..37: mol_type = other DNA
gagaaattaactatgcacattgacaacattgaaaacc

SEQ ID NO: 204 - DNA, 42 bp, synthetic construct
  source 1..42: mol_type = other DNA
catggtatatctccttcttattaggcgaaggaggttgtcagt

SEQ ID NO: 205 - DNA, 38 bp, synthetic construct
  source 1..38: mol_type = other DNA
cgaaggtaacctgttcatggtatatctccttcttatta

SEQ ID NO: 206 - DNA, 19 bp, synthetic construct
  source 1..19: mol_type = other DNA
aacaggttaccttcgagcg

SEQ ID NO: 207 - protein, 493 aa, Xanthomonas campestris
MHALPSIATPTTATPAWHGCIFNGDWVPGSGGTLQIHEPATGGLLHEVGKADLSDVEAAIAQAKHAQRAWATTSPRERAAVFHRAAQLMEAHRAEATLLIARETGGIMPKAEREVGEAIAYYQQAAGLPLQAMGQVLPTAAGQLSLARHLPLGIIAVISPFNFPLILSLRSVAPALAMGNAVILKPDPRTPYTGGVIIAQVLEEAGLPKGLLHVLHGGADIGQALVEAPDVPMIAFTGSTAAGRRIGELAGRHLKKVALELGGNNAVIVLDDADLERAASAIAFGAYLHQGQICMATGRVLVQRGVADALTKLLADKARHLPVGDPVSGTVALGPIIDQRQLQRVLDIVDDSIDAGAVVEAGATHDGLFYAATVLSNVRPGMRVFDEEVFGPVINITVFDTDEEAAVLANHGEYGLVAGIMSASVSRAMVLGEQLHTGLLHINDQTVADEVINPFGGTGASGNGTSVGGPADWEQYMHWQWLTIKHAVPQYPF

SEQ ID NO: 208 - DNA, 1482 bp, Xanthomonas campestris
  source 1..1482: mol_type = other DNA
atgcatgcgctccccagcattgcgacacccacgaccgccacaccggcgtggcacggctgtatcttcaatggcgactgggttcccggtagcggcggcacgctgcagatccatgagccggctaccggcggcctgttgcacgaggtcggcaaggccgatctatccgatgtggaggccgccattgcgcaggccaagcatgcccaacgtgcctgggcaaccacctcgccgcgcgagcgtgcagcggtgttccaccgcgctgcgcaactgatggaagcgcaccgcgccgaggccaccttgctgatcgcgcgcgagaccggcggcatcatgcccaaggccgagcgcgaggtgggcgaggcgattgcctactaccagcaagcggccgggctgccgctgcaggcgatgggccaggtgctgccaaccgccgcaggccagctcagcctggccaggcatctgccgctgggcatcattgcggtgatttcgcccttcaacttcccgctgatcctgtcgctgcggtcggtggcaccggcgctggcgatgggcaatgcggtgatcctcaagccggacccgcgcacgccgtataccggcggtgtgatcatcgcccaagtgctcgaagaagccgggctgcccaaggggctgctgcacgtgctgcatggcggcgccgacatcgggcaggcactggtcgaagcgccggatgtgccgatgattgccttcaccggctccaccgccgccgggcgccggatcggcgagctcgccggccgtcacttgaaaaaggtagcgctggagctcggcggcaataacgcagtgatcgtgctcgacgacgccgacctggagcgcgccgcatcggcgatcgccttcggtgcgtacctgcatcaaggccagatctgcatggccaccggccgcgtgttggtgcaacgcggcgtggccgacgcgctgaccaaactgctggccgacaaggcacgccacctgccggtgggtgacccggtcagcggcacggtggcgctgggcccgatcatcgaccagcgccagttgcagcgcgtgctggacatcgtcgatgacagcatcgacgccggcgcggtggtcgaagccggcgccacccacgacggcctgttctacgcagcgaccgtgttgtcgaacgtgcgcccgggcatgcgggtgttcgatgaggaagtgttcggcccggtgatcaacatcacggtgttcgataccgacgaagaagccgcggtactcgccaatcacggcgaatacggcctggtggcaggcatcatgtcggcatcggtgtcgcgcgccatggtgctgggtgagcaattgcacaccggcctgctgcacatcaacgaccagaccgtggccgatgaggtcatcaatccattcggtggcacgggcgcctctggcaacggcaccagcgtgggtgggccggccgattgggagcagtacatgcactggcagtggctgacgatcaagcacgcggtgcctcagtacccgttctga

SEQ ID NO: 209 - DNA, 34 bp, synthetic construct
  source 1..34: mol_type = other DNA
caccatcacggatcccatgcgctccccagcattg

SEQ ID NO: 210 - DNA, 34 bp, synthetic construct
  source 1..34: mol_type = other DNA
cagctaattaagctttcagaacgggtactgaggc